European Patent Specification EP 4 118 200 B1, published October 8, 2025. Title: POLYPEPTIDE. Applicant: Freeline Therapeutics Limited. The sequence listing filed with the application follows.

SEQUENCE LISTING (64 sequences)

SEQ ID NO: 1 - protein, 536 aa, Homo sapiens
MEFSSPSREECPKPLSRVSIMAGSLTGLLLLQAVSWASGARPCIPKSFGYSSVVCVCNATYCDSFDPPTFPALGTFSRYESTRSGRRMELSMGPIQANHTGTGLLLTLQPEQKFQKVKGFGGAMTDAAALNILALSPPAQNLLLKSYFSEEGIGYNIIRVPMASCDFSIRTYTYADTPDDFQLHNFSLPEEDTKLKIPLIHRALQLAQRPVSLLASPWTSPTWLKTNGAVNGKGSLKGQPGDIYHQTWARYFVKFLDAYAEHKLQFWAVTAENEPSAGLLSGYPFQCLGFTPEHQRDFIARDLGPTLANSTHHNVRLLMLDDQRLLLPHWAKVVLTDPEAAKYVHGIAVHWYLDFLAPAKATLGETHRLFPNTMLFASEACVGSKFWEQSVRLGSWDRGMQYSHSIITNLLYHVVGWTDWNLALNPEGGPNWVRNFVDSPIIVDITKDTFYKQPMFYHLGHFSKFIPEGSQRVGLVASQKNDLDAVALMHPDGSAVVVVLNRSSKDVPLTIKDPAVGFLETISPGYSIHTYLWRRQ

SEQ ID NO: 2 - protein, 497 aa, Homo sapiens
ARPCIPKSFGYSSVVCVCNATYCDSFDPPTFPALGTFSRYESTRSGRRMELSMGPIQANHTGTGLLLTLQPEQKFQKVKGFGGAMTDAAALNILALSPPAQNLLLKSYFSEEGIGYNIIRVPMASCDFSIRTYTYADTPDDFQLHNFSLPEEDTKLKIPLIHRALQLAQRPVSLLASPWTSPTWLKTNGAVNGKGSLKGQPGDIYHQTWARYFVKFLDAYAEHKLQFWAVTAENEPSAGLLSGYPFQCLGFTPEHQRDFIARDLGPTLANSTHHNVRLLMLDDQRLLLPHWAKVVLTDPEAAKYVHGIAVHWYLDFLAPAKATLGETHRLFPNTMLFASEACVGSKFWEQSVRLGSWDRGMQYSHSIITNLLYHVVGWTDWNLALNPEGGPNWVRNFVDSPIIVDITKDTFYKQPMFYHLGHFSKFIPEGSQRVGLVASQKNDLDAVALMHPDGSAVVVVLNRSSKDVPLTIKDPAVGFLETISPGYSIHTYLWRRQ

SEQ ID NO: 3 - protein, 497 aa, Artificial Sequence; identical to SEQ ID NO: 2
  VPRIV

SEQ ID NO: 4 - protein, 536 aa, Artificial Sequence
  Synthetic GCase protein
MEFSSPSREECPKPLSRVSIMAGSLTGLLLLQAVSWASGARPCIPKSFGYSSVVCVCNATYCDSFDPPTFPALGTFSRYESTRSGRRMELSMGPIQANHTGTGLLLTLQPEQKFQKVKGFGGAMTDAAALNILALSPPAQNLLLKSYFSEEGIGYNIIRVPMASCDFSIRTYTYADTPDDFQLLNFSLPEEDTKLKIPLIHRALQLAQRPVSLLASPWTSPTWLKTNGAVNGKGSLKGQPGDIYHQTWARYFVKFLDAYAEHKLQFWAVTAENEPSAGLLSGYPFQCLGFTPEHQRDFIARDLGPTLANSTHHNVRLLMLDDQRLLLPHWAKVVLTDPEAAKYVHGIAVHWYLDFLAPAKATLGETHRLFPNTMLFASEACVGSKFWEQSVRLGSWDRGMQYSHSIITNLLYHVVGWTDWNLALNPEGGPNWVRNFVDSPIIVDITKDTFYKQPMFYHLGHFSKFIPEGSQRVGLVASQKNDLDAVALMHPDGSAVVVVLNRSSKDVPLTIKDPAVGFLETISPGYSIHTYLWRRQ

SEQ ID NO: 5 - protein, 536 aa, Artificial Sequence
  Synthetic GCase protein
MEFSSPSREECPKPLSRVSIMAGSLTGLLLLQAVSWASGARPCIPKSFGYSSVVCVCNATYCDSFDPPTFPALGTFSRYESTRSGRRMELSMGPIQANHTGTGLLLTLQPEQKFQKVKGFGGAMTDAAALNILALSPPAQNLLLKSYFSEEGIGYNIIRVPMASCDFSIRTYTYADTPDDFQLLNFSLPEEDTKLKIPLIHRALQLAQRPVSLLASPWTSPTWLKTNGAVNGKGSLKGQPGDIYHQTWARYFVKFLDAYAEHKLQFWAVTAENEPSAGLLSGYPFQCLGFTPEHQRDFIARDLGPTLANSTHHNVRLLMLDDQRLLLPHWAKVVLTDPEAAKYVHGIAVHWYLDFLAPANATLGETHRLFPNTMLFASEACVGSKFWEQSVRLGSWDRGMQYSHSIITNLLYHVVGWTDWNLALNPEGGPNWVRNFVDSPIIVDITKDTFYKQPMFYHLGHFSKFIPEGSQRVGLVASQKNDLDAVALMHPDGSAVVVVLNRSSKDVPLTIKDPAVGFLETISPGYSIHTYLWRRQ

SEQ ID NO: 6 - DNA, 1494 bp, Artificial Sequence
  Synthetic construct
gccaggccctgcatccctaagagctttggctacagctctgtggtgtgtgtgtgcaatgccacctactgtgacagctttgacccccccacctttcctgccctgggcaccttcagcagatatgagagcaccaggtctgggaggaggatggagctgagcatggggcccatccaggctaatcacactggcactggcctgctgctgaccctgcagcctgagcagaagttccagaaagtaaagggctttggaggggccatgactgatgctgctgctctgaacatcctggccctgagcccccctgcccagaatctgctgctgaagagctacttctctgaggagggcattggctataacatcatcagggtgcccatggccagctgtgacttcagcatcaggacctacacctatgctgacacccctgatgatttccagctgcacaacttcagcctgcctgaggaggataccaagctgaagatcccactgatccacagggctctgcagctggcccagaggcctgtgagcctgctggccagcccctggaccagccccacttggctgaagaccaatggggctgtgaatgggaaggggagcctgaagggacagcctggagacatctaccaccagacctgggccagatactttgtgaagttcctggatgcctatgctgagcacaagctgcagttctgggctgtgactgctcagaatgagccttctgctgggctgctgtctggctaccccttccaatgcctgggcttcacccctgagcatcagagggacttcattgccagggacctgggccctaccctggccaacagcactcaccataatgttaggctgctgatgctggatgaccagaggctgctgctgccccactgggctaaggtggtgctgactgaccctgaggctgctaaatatgtgcatggcattgctgtgcattggtacctggactttctggctcctgccaaggccaccctgggggagacccacaggctgttccccaacaccatgctgtttgcctctgaggcctgtgtgggcagcaagttctgggagcagtctgtgaggctgggcagctgggatagggggatgcagtacagccacagcatcatcaccaacctgctgtaccatgtggtgggctggactgactggaacctggccctgaaccctgagggaggacctaactgggtcagaaactttgtggacagccccatcattgtggacatcaccaaggacaccttttacaagcagcccatgttctaccacctgggccacttcagcaagttcatccctgagggcagccagagagtggggctggtggccagccagaagaatgacctggatgctgtggctctgatgcatcctgatggctctgctgtggtggtggtgctgaacaggagctctaaggatgtgcctctgaccatcaaggatcctgctgtgggcttcctggagaccatcagccctggctacagcatccacacctacctgtggaggaggcagtga

SEQ ID NO: 7 - DNA, 1494 bp, Artificial Sequence
  Synthetic construct
gccaggccctgtatccctaagagctttggctacagctcagtagtttgtgtctgtaatgccacatactgtgactcctttgacccccctaccttccctgccctgggaaccttcagcagatatgagtcaacaagatcaggaaggaggatggagctgtcaatgggacccatccaggctaatcacacaggcacaggcctgctgctgaccctgcagccagaacagaagttccagaaagtgaagggatttggaggagccatgacagatgctgctgctctcaacatcctggccctgtcaccccctgcccagaatctgctgctgaagtcatacttctctgaagaaggaattggatataacatcatcagggtgcccatggccagctgtgacttctccatcaggacctacacctatgctgacacccctgatgatttccagctgcacaacttcagcctcccagaggaagataccaagctcaagatccctctgatacatagggcactgcagctggcccagaggcctgtgtcactcctggccagcccctggacatcacccacttggctcaagaccaatggagctgtgaatggaaagggatcactcaagggacagcctggagacatctaccaccagacctgggccagatactttgtgaagttcctggatgcctatgctgagcacaagctgcagttctgggcagtgacagctcagaatgagccttctgctggactgctgtcaggataccccttccagtgtctgggcttcacccctgaacatcagagggacttcattgccagggacctgggacctacccttgccaactcaactcaccacaatgtcaggctgctcatgctggatgaccagaggctgctgctgccccactgggccaaggtggtgctgacagacccagaagctgctaaatatgtgcatggcattgctgtgcattggtacctggacttcctggctccagccaaggccaccctgggagagacacacaggctgttccccaacaccatgctctttgcctctgaggcctgtgtgggctccaagttctgggagcagtcagtgaggctgggctcctgggataggggaatgcagtacagccacagcatcatcacaaacctcctgtaccatgtggtgggctggactgactggaacctggccctgaaccctgaaggaggacccaactgggtcagaaattttgtggactcacccatcattgtggacatcaccaaggacacattctacaagcagcccatgttctaccacctgggccacttcagcaagttcatccctgagggctcccagagggtgggactggtggcctcacagaagaatgacctggatgcagtggccctgatgcatcctgatggctctgctgtggtggttgtgctgaatagatcctctaaggatgtgcctctgaccatcaaggatcctgctgtgggcttcctggagacaatctcacctggctactccatccacacctacctgtggaggaggcagtga

SEQ ID NO: 8 - DNA, 1494 bp, Artificial Sequence
  Synthetic construct
gccaggccctgcatccctaagagctttggctacagctctgtggtgtgtgtgtgcaatgccacatactgtgactcctttgacccccccacctttcctgccctgggcacattctccagatatgagagcacaagatctgggagaaggatggagctgagcatggggcccatccaggctaatcacactggcacaggcctgctgctgaccctgcagcctgaacagaagtttcagaaagtgaagggatttggaggggccatgacagatgctgctgctctgaatatcctggccctgtcaccccctgcccagaatctgctgctgaagagctacttttcagaagaaggaattggatataatatcatcagagtgcccatggccagctgtgacttttccatcagaacctacacctatgcagacacccctgatgattttcagctgcacaattttagcctgcctgaggaagataccaagctgaagatacccctgattcacagggccctgcagctggcccagaggcctgtttcactgctggccagcccctggacatcacccacctggctgaagaccaatggagctgtgaatgggaaggggtcactgaagggacagcctggagacatctaccaccagacctgggccagatactttgtgaagtttctggatgcctatgctgagcacaagctgcagttttgggcagtgacagctcagaatgagccttcagctgggctgctgtcaggatacccctttcagtgcctgggctttacccctgaacatcagagggactttattgccagggacctgggccctaccctggccaatagcacccaccataatgtgaggttgctgatgctggatgaccagaggctgctgctgccccactgggcaaaggtggtgctgacagaccctgaagcagctaaatatgttcatggcattgctgtgcattggtacctggactttctggctcctgccaaggccaccctgggggagacacacaggctgtttcccaataccatgctgtttgcctctgaggcctgtgtgggctccaagttttgggagcagtctgtgaggctgggctcctgggatagagggatgcagtacagccacagcatcatcaccaatctgctgtaccatgtggtgggctggactgactggaatctggccctgaatcctgaaggaggacctaactgggtcaggaattttgtggacagccccatcattgtggacatcaccaaggacaccttttacaagcagcccatgttttaccacctgggccactttagcaagtttattcctgagggctcccagagagtggggctggttgccagccagaagaatgacctggatgcagtggcactgatgcatcctgatggctcagctgttgtggtggtgctgaatagatccagcaaggatgtgcctctgaccatcaaggatcctgctgtgggctttctggagacaatctcacctggctactccattcacacctacctgtggagaaggcagtga

SEQ ID NO: 9 - DNA, 1494 bp, Artificial Sequence
  Synthetic construct
gccaggccttgcatcccaaagtctttcggctacagctccgtggtgtgcgtgtgcaacgccacctattgtgactccttcgatccccctacctttcccgccctgggcacattttctagatacgagtctacacgcagcggccggagaatggagctgagcatgggccctatccaggccaatcacacaggaacaggcctgctgctgaccctgcagccagagcagaagttccagaaggtgaagggctttggcggagccatgacagatgcagccgccctgaacatcctggccctgtccccacccgcccagaatctgctgctgaagtcctacttctctgaggagggcatcggctataacatcatccgggtgcccatggccagctgcgacttttccatcagaacctacacatatgccgatacccctgacgatttccagctgcacaatttttccctgccagaggaggatacaaagctgaagatccccctgattcaccgggccctgcagctggcacagcggcccgtgagcctgctggccagcccctggacctcccctacatggctgaagaccaacggcgccgtgaatggcaagggctctctgaagggacagcctggcgacatctaccaccagacatgggccagatatttcgtgaagtttctggatgcctacgccgagcacaagctgcagttctgggccgtgacagcacagaatgagccttctgccggcctgctgagcggctatcccttccagtgcctgggctttacacctgagcaccagcgggactttatcgccagagatctgggcccaaccctggccaactccacacaccacaatgtgaggctgctgatgctggacgatcagcgcctgctgctgcctcactgggccaaggtggtgctgaccgacccagaggccgccaagtacgtgcacggcatcgccgtgcactggtatctggatttcctggcacctgcaaaggccaccctgggagagacacaccggctgttccctaacaccatgctgtttgccagcgaggcctgcgtgggctccaagttttgggagcagtccgtgaggctgggatcttgggacagaggcatgcagtactcccactctatcatcaccaatctgctgtatcacgtggtgggctggacagactggaacctggccctgaatccagagggcggccccaactgggtgagaaatttcgtggatagccccatcatcgtggacatcaccaaggatacattctacaagcagccaatgttttatcacctgggccacttctctaagtttatccctgagggcagccagagggtgggcctggtggccagccagaagaacgacctggatgccgtggccctgatgcaccctgatggctccgccgtggtggtggtgctgaatcgctctagcaaggacgtgcctctgaccatcaaggatccagccgtgggatttctggagactatttcacctggctattcaattcatacctacctgtggaggaggcagtga

SEQ ID NO: 10 - DNA, 1611 bp, Artificial Sequence
  Synthetic construct
atggagttttcaagtccttccagagaggaatgtcccaagcctttgagtagggtaagcatcatggctggcagcctcacaggattgcttctacttcaggcagtgtcgtgggcatcaggtgccaggccctgcatccctaagagctttggctacagctctgtggtgtgtgtgtgcaatgccacctactgtgacagctttgacccccccacctttcctgccctgggcaccttcagcagatatgagagcaccaggtctgggaggaggatggagctgagcatggggcccatccaggctaatcacactggcactggcctgctgctgaccctgcagcctgagcagaagttccagaaagtaaagggctttggaggggccatgactgatgctgctgctctgaacatcctggccctgagcccccctgcccagaatctgctgctgaagagctacttctctgaggagggcattggctataacatcatcagggtgcccatggccagctgtgacttcagcatcaggacctacacctatgctgacacccctgatgatttccagctgcacaacttcagcctgcctgaggaggataccaagctgaagatcccactgatccacagggctctgcagctggcccagaggcctgtgagcctgctggccagcccctggaccagccccacttggctgaagaccaatggggctgtgaatgggaaggggagcctgaagggacagcctggagacatctaccaccagacctgggccagatactttgtgaagttcctggatgcctatgctgagcacaagctgcagttctgggctgtgactgctcagaatgagccttctgctgggctgctgtctggctaccccttccaatgcctgggcttcacccctgagcatcagagggacttcattgccagggacctgggccctaccctggccaacagcactcaccataatgttaggctgctgatgctggatgaccagaggctgctgctgccccactgggctaaggtggtgctgactgaccctgaggctgctaaatatgtgcatggcattgctgtgcattggtacctggactttctggctcctgccaaggccaccctgggggagacccacaggctgttccccaacaccatgctgtttgcctctgaggcctgtgtgggcagcaagttctgggagcagtctgtgaggctgggcagctgggatagggggatgcagtacagccacagcatcatcaccaacctgctgtaccatgtggtgggctggactgactggaacctggccctgaaccctgagggaggacctaactgggtcagaaactttgtggacagccccatcattgtggacatcaccaaggacaccttttacaagcagcccatgttctaccacctgggccacttcagcaagttcatccctgagggcagccagagagtggggctggtggccagccagaagaatgacctggatgctgtggctctgatgcatcctgatggctctgctgtggtggtggtgctgaacaggagctctaaggatgtgcctctgaccatcaaggatcctgctgtgggcttcctggagaccatcagccctggctacagcatccacacctacctgtggaggaggcagtga

SEQ ID NO: 11 - DNA, 1611 bp, Artificial Sequence
  Synthetic construct
atggagttttcaagtccttccagagaggaatgtcccaagcctttgagtagggtaagcatcatggctggcagcctcacaggattgcttctacttcaggcagtgtcgtgggcatcaggtgccaggccctgtatccctaagagctttggctacagctcagtagtttgtgtctgtaatgccacatactgtgactcctttgacccccctaccttccctgccctgggaaccttcagcagatatgagtcaacaagatcaggaaggaggatggagctgtcaatgggacccatccaggctaatcacacaggcacaggcctgctgctgaccctgcagccagaacagaagttccagaaagtgaagggatttggaggagccatgacagatgctgctgctctcaacatcctggccctgtcaccccctgcccagaatctgctgctgaagtcatacttctctgaagaaggaattggatataacatcatcagggtgcccatggccagctgtgacttctccatcaggacctacacctatgctgacacccctgatgatttccagctgcacaacttcagcctcccagaggaagataccaagctcaagatccctctgatacatagggcactgcagctggcccagaggcctgtgtcactcctggccagcccctggacatcacccacttggctcaagaccaatggagctgtgaatggaaagggatcactcaagggacagcctggagacatctaccaccagacctgggccagatactttgtgaagttcctggatgcctatgctgagcacaagctgcagttctgggcagtgacagctcagaatgagccttctgctggactgctgtcaggataccccttccagtgtctgggcttcacccctgaacatcagagggacttcattgccagggacctgggacctacccttgccaactcaactcaccacaatgtcaggctgctcatgctggatgaccagaggctgctgctgccccactgggccaaggtggtgctgacagacccagaagctgctaaatatgtgcatggcattgctgtgcattggtacctggacttcctggctccagccaaggccaccctgggagagacacacaggctgttccccaacaccatgctctttgcctctgaggcctgtgtgggctccaagttctgggagcagtcagtgaggctgggctcctgggataggggaatgcagtacagccacagcatcatcacaaacctcctgtaccatgtggtgggctggactgactggaacctggccctgaaccctgaaggaggacccaactgggtcagaaattttgtggactcacccatcattgtggacatcaccaaggacacattctacaagcagcccatgttctaccacctgggccacttcagcaagttcatccctgagggctcccagagggtgggactggtggcctcacagaagaatgacctggatgcagtggccctgatgcatcctgatggctctgctgtggtggttgtgctgaatagatcctctaaggatgtgcctctgaccatcaaggatcctgctgtgggcttcctggagacaatctcacctggctactccatccacacctacctgtggaggaggcagtga

SEQ ID NO: 12 - DNA, 1611 bp, Artificial Sequence
  Synthetic construct
atggagttttcaagtccttccagagaggaatgtcccaagcctttgagtagggtaagcatcatggctggcagcctcacaggattgcttctacttcaggcagtgtcgtgggcatcaggtgccaggccctgcatccctaagagctttggctacagctctgtggtgtgtgtgtgcaatgccacatactgtgactcctttgacccccccacctttcctgccctgggcacattctccagatatgagagcacaagatctgggagaaggatggagctgagcatggggcccatccaggctaatcacactggcacaggcctgctgctgaccctgcagcctgaacagaagtttcagaaagtgaagggatttggaggggccatgacagatgctgctgctctgaatatcctggccctgtcaccccctgcccagaatctgctgctgaagagctacttttcagaagaaggaattggatataatatcatcagagtgcccatggccagctgtgacttttccatcagaacctacacctatgcagacacccctgatgattttcagctgcacaattttagcctgcctgaggaagataccaagctgaagatacccctgattcacagggccctgcagctggcccagaggcctgtttcactgctggccagcccctggacatcacccacctggctgaagaccaatggagctgtgaatgggaaggggtcactgaagggacagcctggagacatctaccaccagacctgggccagatactttgtgaagtttctggatgcctatgctgagcacaagctgcagttttgggcagtgacagctcagaatgagccttcagctgggctgctgtcaggatacccctttcagtgcctgggctttacccctgaacatcagagggactttattgccagggacctgggccctaccctggccaatagcacccaccataatgtgaggttgctgatgctggatgaccagaggctgctgctgccccactgggcaaaggtggtgctgacagaccctgaagcagctaaatatgttcatggcattgctgtgcattggtacctggactttctggctcctgccaaggccaccctgggggagacacacaggctgtttcccaataccatgctgtttgcctctgaggcctgtgtgggctccaagttttgggagcagtctgtgaggctgggctcctgggatagagggatgcagtacagccacagcatcatcaccaatctgctgtaccatgtggtgggctggactgactggaatctggccctgaatcctgaaggaggacctaactgggtcaggaattttgtggacagccccatcattgtggacatcaccaaggacaccttttacaagcagcccatgttttaccacctgggccactttagcaagtttattcctgagggctcccagagagtggggctggttgccagccagaagaatgacctggatgcagtggcactgatgcatcctgatggctcagctgttgtggtggtgctgaatagatccagcaaggatgtgcctctgaccatcaaggatcctgctgtgggctttctggagacaatctcacctggctactccattcacacctacctgtggagaaggcagtga

SEQ ID NO: 13 - DNA, 1611 bp, Artificial Sequence
  Synthetic construct
atggagttttcaagtccttccagagaggaatgtcccaagcctttgagtagggtaagcatcatggctggcagcctcacaggattgcttctacttcaggcagtgtcgtgggcatcaggtgccaggccttgcatcccaaagtctttcggctacagctccgtggtgtgcgtgtgcaacgccacctattgtgactccttcgatccccctacctttcccgccctgggcacattttctagatacgagtctacacgcagcggccggagaatggagctgagcatgggccctatccaggccaatcacacaggaacaggcctgctgctgaccctgcagccagagcagaagttccagaaggtgaagggctttggcggagccatgacagatgcagccgccctgaacatcctggccctgtccccacccgcccagaatctgctgctgaagtcctacttctctgaggagggcatcggctataacatcatccgggtgcccatggccagctgcgacttttccatcagaacctacacatatgccgatacccctgacgatttccagctgcacaatttttccctgccagaggaggatacaaagctgaagatccccctgattcaccgggccctgcagctggcacagcggcccgtgagcctgctggccagcccctggacctcccctacatggctgaagaccaacggcgccgtgaatggcaagggctctctgaagggacagcctggcgacatctaccaccagacatgggccagatatttcgtgaagtttctggatgcctacgccgagcacaagctgcagttctgggccgtgacagcacagaatgagccttctgccggcctgctgagcggctatcccttccagtgcctgggctttacacctgagcaccagcgggactttatcgccagagatctgggcccaaccctggccaactccacacaccacaatgtgaggctgctgatgctggacgatcagcgcctgctgctgcctcactgggccaaggtggtgctgaccgacccagaggccgccaagtacgtgcacggcatcgccgtgcactggtatctggatttcctggcacctgcaaaggccaccctgggagagacacaccggctgttccctaacaccatgctgtttgccagcgaggcctgcgtgggctccaagttttgggagcagtccgtgaggctgggatcttgggacagaggcatgcagtactcccactctatcatcaccaatctgctgtatcacgtggtgggctggacagactggaacctggccctgaatccagagggcggccccaactgggtgagaaatttcgtggatagccccatcatcgtggacatcaccaaggatacattctacaagcagccaatgttttatcacctgggccacttctctaagtttatccctgagggcagccagagggtgggcctggtggccagccagaagaacgacctggatgccgtggccctgatgcaccctgatggctccgccgtggtggtggtgctgaatcgctctagcaaggacgtgcctctgaccatcaaggatccagccgtgggatttctggagactatttcacctggctattcaattcatacctacctgtggaggaggcagtga

SEQ ID NO: 14 - DNA, 1494 bp, Artificial Sequence
  Synthetic construct
gccaggccctgcatccctaagagctttggctacagctctgtggtgtgtgtgtgcaatgccacctactgtgacagctttgacccccccacctttcctgccctgggcaccttcagcagatatgagagcaccaggtctgggaggaggatggagctgagcatggggcccatccaggctaatcacactggcactggcctgctgctgaccctgcagcctgagcagaagttccagaaagtaaagggctttggaggggccatgactgatgctgctgctctgaacatcctggccctgagcccccctgcccagaatctgctgctgaagagctacttctctgaggagggcattggctataacatcatcagggtgcccatggccagctgtgacttcagcatcaggacctacacctatgctgacacccctgatgatttccagctgcacaacttcagcctgcctgaggaggataccaagctgaagatcccactgatccacagggctctgcagctggcccagaggcctgtgagcctgctggccagcccctggaccagccccacttggctgaagaccaatggggctgtgaatgggaaggggagcctgaagggacagcctggagacatctaccaccagacctgggccagatactttgtgaagttcctggatgcctatgctgagcacaagctgcagttctgggctgtgactgctgagaatgagccttctgctgggctgctgtctggctaccccttccaatgcctgggcttcacccctgagcatcagagggacttcattgccagggacctgggccctaccctggccaacagcactcaccataatgttaggctgctgatgctggatgaccagaggctgctgctgccccactgggctaaggtggtgctgactgaccctgaggctgctaaatatgtgcatggcattgctgtgcattgctacctggactttctggctcctgccaaggccaccctgggggagacccacaggctgttccccaacaccatgctgtttgcctctgagtgctgtgtgggcagcaagttctgggagcagtctgtgaggctgggcagctgggatagggggatgcagtacagccacagcatcatcaccaacctgctgtaccatgtggtgggctggactgactggaacctggccctgaaccctgagggaggacctaactgggtcagaaactttgtggacagccccatcattgtggacatcaccaaggacaccttttacaagcagcccatgttctaccacctgggccacttcagcaagttcatccctgagggcagccagagagtggggctggtggccagccagaagaatgacctggatgctgtggctctgatgcatcctgatggctctgctgtggtggtggtgctgaacaggagctctaaggatgtgcctctgaccatcaaggatcctgctgtgggcttcctggagaccatcagccctggctacagcatccacacctacctgtggaggaggcagtga

SEQ ID NO: 15 - DNA, 1494 bp, Artificial Sequence
  Synthetic construct
gccaggccctgtatccctaagagctttggctacagctcagtagtttgtgtctgtaatgccacatactgtgactcctttgacccccctaccttccctgccctgggaaccttcagcagatatgagtcaacaagatcaggaaggaggatggagctgtcaatgggacccatccaggctaatcacacaggcacaggcctgctgctgaccctgcagccagaacagaagttccagaaagtgaagggatttggaggagccatgacagatgctgctgctctcaacatcctggccctgtcaccccctgcccagaatctgctgctgaagtcatacttctctgaagaaggaattggatataacatcatcagggtgcccatggccagctgtgacttctccatcaggacctacacctatgctgacacccctgatgatttccagctgcacaacttcagcctcccagaggaagataccaagctcaagatccctctgatacatagggcactgcagctggcccagaggcctgtgtcactcctggccagcccctggacatcacccacttggctcaagaccaatggagctgtgaatggaaagggatcactcaagggacagcctggagacatctaccaccagacctgggccagatactttgtgaagttcctggatgcctatgctgagcacaagctgcagttctgggcagtgacagctgaaaatgagccttctgctggactgctgtcaggataccccttccagtgtctgggcttcacccctgaacatcagagggacttcattgccagggacctgggacctacccttgccaactcaactcaccacaatgtcaggctgctcatgctggatgaccagaggctgctgctgccccactgggccaaggtggtgctgacagacccagaagctgctaaatatgtgcatggcattgctgtgcattgctacctggacttcctggctccagccaaggccaccctgggagagacacacaggctgttccccaacaccatgctctttgcctctgagtgctgtgtgggctccaagttctgggagcagtcagtgaggctgggctcctgggataggggaatgcagtacagccacagcatcatcacaaacctcctgtaccatgtggtgggctggactgactggaacctggccctgaaccctgaaggaggacccaactgggtcagaaattttgtggactcacccatcattgtggacatcaccaaggacacattctacaagcagcccatgttctaccacctgggccacttcagcaagttcatccctgagggctcccagagggtgggactggtggcctcacagaagaatgacctggatgcagtggccctgatgcatcctgatggctctgctgtggtggttgtgctgaatagatcctctaaggatgtgcctctgaccatcaaggatcctgctgtgggcttcctggagacaatctcacctggctactccatccacacctacctgtggaggaggcagtga

SEQ ID NO: 16 - DNA, 1494 bp, Artificial Sequence
  Synthetic construct
gccaggccctgcatccctaagagctttggctacagctctgtggtgtgtgtgtgcaatgccacatactgtgactcctttgacccccccacctttcctgccctgggcacattctccagatatgagagcacaagatctgggagaaggatggagctgagcatggggcccatccaggctaatcacactggcacaggcctgctgctgaccctgcagcctgaacagaagtttcagaaagtgaagggatttggaggggccatgacagatgctgctgctctgaatatcctggccctgtcaccccctgcccagaatctgctgctgaagagctacttttcagaagaaggaattggatataatatcatcagagtgcccatggccagctgtgacttttccatcagaacctacacctatgcagacacccctgatgattttcagctgcacaattttagcctgcctgaggaagataccaagctgaagatacccctgattcacagggccctgcagctggcccagaggcctgtttcactgctggccagcccctggacatcacccacctggctgaagaccaatggagctgtgaatgggaaggggtcactgaagggacagcctggagacatctaccaccagacctgggccagatactttgtgaagtttctggatgcctatgctgagcacaagctgcagttttgggcagtgacagctgaaaatgagccttcagctgggctgctgtcaggatacccctttcagtgcctgggctttacccctgaacatcagagggactttattgccagggacctgggccctaccctggccaatagcacccaccataatgtgaggttgctgatgctggatgaccagaggctgctgctgccccactgggcaaaggtggtgctgacagaccctgaagcagctaaatatgttcatggcattgctgtgcattgctacctggactttctggctcctgccaaggccaccctgggggagacacacaggctgtttcccaataccatgctgtttgcctctgagtgctgtgtgggctccaagttttgggagcagtctgtgaggctgggctcctgggatagagggatgcagtacagccacagcatcatcaccaatctgctgtaccatgtggtgggctggactgactggaatctggccctgaatcctgaaggaggacctaactgggtcaggaattttgtggacagccccatcattgtggacatcaccaaggacaccttttacaagcagcccatgttttaccacctgggccactttagcaagtttattcctgagggctcccagagagtggggctggttgccagccagaagaatgacctggatgcagtggcactgatgcatcctgatggctcagctgttgtggtggtgctgaatagatccagcaaggatgtgcctctgaccatcaaggatcctgctgtgggctttctggagacaatctcacctggctactccattcacacctacctgtggagaaggcagtga

SEQ ID NO: 17 - DNA, 1494 bp, Artificial Sequence
  Synthetic construct
gccaggccttgcatcccaaagtctttcggctacagctccgtggtgtgcgtgtgcaacgccacctattgtgactccttcgatccccctacctttcccgccctgggcacattttctagatacgagtctacacgcagcggccggagaatggagctgagcatgggccctatccaggccaatcacacaggaacaggcctgctgctgaccctgcagccagagcagaagttccagaaggtgaagggctttggcggagccatgacagatgcagccgccctgaacatcctggccctgtccccacccgcccagaatctgctgctgaagtcctacttctctgaggagggcatcggctataacatcatccgggtgcccatggccagctgcgacttttccatcagaacctacacatatgccgatacccctgacgatttccagctgcacaatttttccctgccagaggaggatacaaagctgaagatccccctgattcaccgggccctgcagctggcacagcggcccgtgagcctgctggccagcccctggacctcccctacatggctgaagaccaacggcgccgtgaatggcaagggctctctgaagggacagcctggcgacatctaccaccagacatgggccagatatttcgtgaagtttctggatgcctacgccgagcacaagctgcagttctgggccgtgacagcagagaatgagccttctgccggcctgctgagcggctatcccttccagtgcctgggctttacacctgagcaccagcgggactttatcgccagagatctgggcccaaccctggccaactccacacaccacaatgtgaggctgctgatgctggacgatcagcgcctgctgctgcctcactgggccaaggtggtgctgaccgacccagaggccgccaagtacgtgcacggcatcgccgtgcactgctatctggatttcctggcacctgcaaaggccaccctgggagagacacaccggctgttccctaacaccatgctgtttgccagcgagtgctgcgtgggctccaagttttgggagcagtccgtgaggctgggatcttgggacagaggcatgcagtactcccactctatcatcaccaatctgctgtatcacgtggtgggctggacagactggaacctggccctgaatccagagggcggccccaactgggtgagaaatttcgtggatagccccatcatcgtggacatcaccaaggatacattctacaagcagccaatgttttatcacctgggccacttctctaagtttatccctgagggcagccagagggtgggcctggtggccagccagaagaacgacctggatgccgtggccctgatgcaccctgatggctccgccgtggtggtggtgctgaatcgctctagcaaggacgtgcctctgaccatcaaggatccagccgtgggatttctggagactatttcacctggctattcaattcatacctacctgtggaggaggcagtga

SEQ ID NO: 18 - DNA, 1611 bp, Artificial Sequence
  Synthetic construct
atggagttttcaagtccttccagagaggaatgtcccaagcctttgagtagggtaagcatcatggctggcagcctcacaggattgcttctacttcaggcagtgtcgtgggcatcaggtgccaggccctgcatccctaagagctttggctacagctctgtggtgtgtgtgtgcaatgccacctactgtgacagctttgacccccccacctttcctgccctgggcaccttcagcagatatgagagcaccaggtctgggaggaggatggagctgagcatggggcccatccaggctaatcacactggcactggcctgctgctgaccctgcagcctgagcagaagttccagaaagtaaagggctttggaggggccatgactgatgctgctgctctgaacatcctggccctgagcccccctgcccagaatctgctgctgaagagctacttctctgaggagggcattggctataacatcatcagggtgcccatggccagctgtgacttcagcatcaggacctacacctatgctgacacccctgatgatttccagctgcacaacttcagcctgcctgaggaggataccaagctgaagatcccactgatccacagggctctgcagctggcccagaggcctgtgagcctgctggccagcccctggaccagccccacttggctgaagaccaatggggctgtgaatgggaaggggagcctgaagggacagcctggagacatctaccaccagacctgggccagatactttgtgaagttcctggatgcctatgctgagcacaagctgcagttctgggctgtgactgctgagaatgagccttctgctgggctgctgtctggctaccccttccaatgcctgggcttcacccctgagcatcagagggacttcattgccagggacctgggccctaccctggccaacagcactcaccataatgttaggctgctgatgctggatgaccagaggctgctgctgccccactgggctaaggtggtgctgactgaccctgaggctgctaaatatgtgcatggcattgctgtgcattgctacctggactttctggctcctgccaaggccaccctgggggagacccacaggctgttccccaacaccatgctgtttgcctctgagtgctgtgtgggcagcaagttctgggagcagtctgtgaggctgggcagctgggatagggggatgcagtacagccacagcatcatcaccaacctgctgtaccatgtggtgggctggactgactggaacctggccctgaaccctgagggaggacctaactgggtcagaaactttgtggacagccccatcattgtggacatcaccaaggacaccttttacaagcagcccatgttctaccacctgggccacttcagcaagttcatccctgagggcagccagagagtggggctggtggccagccagaagaatgacctggatgctgtggctctgatgcatcctgatggctctgctgtggtggtggtgctgaacaggagctctaaggatgtgcctctgaccatcaaggatcctgctgtgggcttcctggagaccatcagccctggctacagcatccacacctacctgtggaggaggcagtga

SEQ ID NO: 19 - DNA, 1611 bp, Artificial Sequence
  Synthetic construct
atggagttttcaagtccttccagagaggaatgtcccaagcctttgagtagggtaagcatcatggctggcagcctcacaggattgcttctacttcaggcagtgtcgtgggcatcaggtgccaggccctgtatccctaagagctttggctacagctcagtagtttgtgtctgtaatgccacatactgtgactcctttgacccccctaccttccctgccctgggaaccttcagcagatatgagtcaacaagatcaggaaggaggatggagctgtcaatgggacccatccaggctaatcacacaggcacaggcctgctgctgaccctgcagccagaacagaagttccagaaagtgaagggatttggaggagccatgacagatgctgctgctctcaacatcctggccctgtcaccccctgcccagaatctgctgctgaagtcatacttctctgaagaaggaattggatataacatcatcagggtgcccatggccagctgtgacttctccatcaggacctacacctatgctgacacccctgatgatttccagctgcacaacttcagcctcccagaggaagataccaagctcaagatccctctgatacatagggcactgcagctggcccagaggcctgtgtcactcctggccagcccctggacatcacccacttggctcaagaccaatggagctgtgaatggaaagggatcactcaagggacagcctggagacatctaccaccagacctgggccagatactttgtgaagttcctggatgcctatgctgagcacaagctgcagttctgggcagtgacagctgaaaatgagccttctgctggactgctgtcaggataccccttccagtgtctgggcttcacccctgaacatcagagggacttcattgccagggacctgggacctacccttgccaactcaactcaccacaatgtcaggctgctcatgctggatgaccagaggctgctgctgccccactgggccaaggtggtgctgacagacccagaagctgctaaatatgtgcatggcattgctgtgcattgctacctggacttcctggctccagccaaggccaccctgggagagacacacaggctgttccccaacaccatgctctttgcctctgagtgctgtgtgggctccaagttctgggagcagtcagtgaggctgggctcctgggataggggaatgcagtacagccacagcatcatcacaaacctcctgtaccatgtggtgggctggactgactggaacctggccctgaaccctgaaggaggacccaactgggtcagaaattttgtggactcacccatcattgtggacatcaccaaggacacattctacaagcagcccatgttctaccacctgggccacttcagcaagttcatccctgagggctcccagagggtgggactggtggcctcacagaagaatgacctggatgcagtggccctgatgcatcctgatggctctgctgtggtggttgtgctgaatagatcctctaaggatgtgcctctgaccatcaaggatcctgctgtgggcttcctggagacaatctcacctggctactccatccacacctacctgtggaggaggcagtga

SEQ ID NO: 20 - DNA, 1611 bp, Artificial Sequence
  Synthetic construct
atggagttttcaagtccttccagagaggaatgtcccaagcctttgagtagggtaagcatcatggctggcagcctcacaggattgcttctacttcaggcagtgtcgtgggcatcaggtgccaggccctgcatccctaagagctttggctacagctctgtggtgtgtgtgtgcaatgccacatactgtgactcctttgacccccccacctttcctgccctgggcacattctccagatatgagagcacaagatctgggagaaggatggagctgagcatggggcccatccaggctaatcacactggcacaggcctgctgctgaccctgcagcctgaacagaagtttcagaaagtgaagggatttggaggggccatgacagatgctgctgctctgaatatcctggccctgtcaccccctgcccagaatctgctgctgaagagctacttttcagaagaaggaattggatataatatcatcagagtgcccatggccagctgtgacttttccatcagaacctacacctatgcagacacccctgatgattttcagctgcacaattttagcctgcctgaggaagataccaagctgaagatacccctgattcacagggccctgcagctggcccagaggcctgtttcactgctggccagcccctggacatcacccacctggctgaagaccaatggagctgtgaatgggaaggggtcactgaagggacagcctggagacatctaccaccagacctgggccagatactttgtgaagtttctggatgcctatgctgagcacaagctgcagttttgggcagtgacagctgaaaatgagccttcagctgggctgctgtcaggatacccctttcagtgcctgggctttacccctgaacatcagagggactttattgccagggacctgggccctaccctggccaatagcacccaccataatgtgaggttgctgatgctggatgaccagaggctgctgctgccccactgggcaaaggtggtgctgacagaccctgaagcagctaaatatgttcatggcattgctgtgcattgctacctggactttctggctcctgccaaggccaccctgggggagacacacaggctgtttcccaataccatgctgtttgcctctgagtgctgtgtgggctccaagttttgggagcagtctgtgaggctgggctcctgggatagagggatgcagtacagccacagcatcatcaccaatctgctgtaccatgtggtgggctggactgactggaatctggccctgaatcctgaaggaggacctaactgggtcaggaattttgtggacagccccatcattgtggacatcaccaaggacaccttttacaagcagcccatgttttaccacctgggccactttagcaagtttattcctgagggctcccagagagtggggctggttgccagccagaagaatgacctggatgcagtggcactgatgcatcctgatggctcagctgttgtggtggtgctgaatagatccagcaaggatgtgcctctgaccatcaaggatcctgctgtgggctttctggagacaatctcacctggctactccattcacacctacctgtggagaaggcagtga

SEQ ID NO: 21 - DNA, 1611 bp, Artificial Sequence
  Synthetic construct
atggagttttcaagtccttccagagaggaatgtcccaagcctttgagtagggtaagcatcatggctggcagcctcacaggattgcttctacttcaggcagtgtcgtgggcatcaggtgccaggccttgcatcccaaagtctttcggctacagctccgtggtgtgcgtgtgcaacgccacctattgtgactccttcgatccccctacctttcccgccctgggcacattttctagatacgagtctacacgcagcggccggagaatggagctgagcatgggccctatccaggccaatcacacaggaacaggcctgctgctgaccctgcagccagagcagaagttccagaaggtgaagggctttggcggagccatgacagatgcagccgccctgaacatcctggccctgtccccacccgcccagaatctgctgctgaagtcctacttctctgaggagggcatcggctataacatcatccgggtgcccatggccagctgcgacttttccatcagaacctacacatatgccgatacccctgacgatttccagctgcacaatttttccctgccagaggaggatacaaagctgaagatccccctgattcaccgggccctgcagctggcacagcggcccgtgagcctgctggccagcccctggacctcccctacatggctgaagaccaacggcgccgtgaatggcaagggctctctgaagggacagcctggcgacatctaccaccagacatgggccagatatttcgtgaagtttctggatgcctacgccgagcacaagctgcagttctgggccgtgacagcagagaatgagccttctgccggcctgctgagcggctatcccttccagtgcctgggctttacacctgagcaccagcgggactttatcgccagagatctgggcccaaccctggccaactccacacaccacaatgtgaggctgctgatgctggacgatcagcgcctgctgctgcctcactgggccaaggtggtgctgaccgacccagaggccgccaagtacgtgcacggcatcgccgtgcactgctatctggatttcctggcacctgcaaaggccaccctgggagagacacaccggctgttccctaacaccatgctgtttgccagcgagtgctgcgtgggctccaagttttgggagcagtccgtgaggctgggatcttgggacagaggcatgcagtactcccactctatcatcaccaatctgctgtatcacgtggtgggctggacagactggaacctggccctgaatccagagggcggccccaactgggtgagaaatttcgtggatagccccatcatcgtggacatcaccaaggatacattctacaagcagccaatgttttatcacctgggccacttctctaagtttatccctgagggcagccagagggtgggcctggtggccagccagaagaacgacctggatgccgtggccctgatgcaccctgatggctccgccgtggtggtggtgctgaatcgctctagcaaggacgtgcctctgaccatcaaggatccagccgtgggatttctggagactatttcacctggctattcaattcatacctacctgtggaggaggcagtga

SEQ ID NO: 22 - DNA, 1494 bp, Artificial Sequence
  Synthetic construct
gccaggccctgcatccctaagagctttggctacagctctgtggtgtgtgtgtgcaatgccacctactgtgacagctttgacccccccacctttcctgccctgggcaccttcagcagatatgagagcaccaggtctgggaggaggatggagctgagcatggggcccatccaggctaatcacactggcactggcctgctgctgaccctgcagcctgagcagaagttccagaaagtaaagggctttggaggggccatgactgatgctgctgctctgaacatcctggccctgagcccccctgcccagaatctgctgctgaagagctacttctctgaggagggcattggctataacatcatcagggtgcccatggccagctgtgacttcagcatcaggacctacacctatgctgacacccctgatgatttccagctgcacaacttcagcctgcctgaggaggataccaagctgaagatcccactgatccacagggctctgcagctggcccagaggcctgtgagcctgctggccagcccctggaccagccccacttggctgaagaccaatggggctgtgaatgggaaggggagcctgaagggacagcctggagacatctaccaccagacctgggccagatactttgtgaagttcctggatgcctatgctgagcacaagctgcagttctgggctgtgactgctcagaatgagccttctgctgggctgctgtctggctaccccttccaatgcctgggcttcacccctgagcatcagagggacttcattgccagggacctgggccctaccctggccaacagcactcaccataatgttaggctgctgatgctggatgaccagaggctgctgctgccccactgggctaaggtggtgctgactgaccctgaggctgctaaatatgtgcatggcattgctgtgcattgctacctggactttctggctcctgccaaggccaccctgggggagacccacaggctgttccccaacaccatgctgtttgcctctgagtgctgtgtgggcagcaagttctgggagcagtctgtgaggctgggcagctgggatagggggatgcagtacagccacagcatcatcaccaacctgctgtaccatgtggtgggctggactgactggaacctggccctgaaccctgagggaggacctaactgggtcagaaactttgtggacagccccatcattgtggacatcaccaaggacaccttttacaagcagcccatgttctaccacctgggccacttcagcaagttcatccctgagggcagccagagagtggggctggtggccagccagaagaatgacctggatgctgtggctctgatgcatcctgatggctctgctgtggtggtggtgctgaacaggagctctaaggatgtgcctctgaccatcaaggatcctgctgtgggcttcctggagaccatcagccctggctacagcatccacacctacctgtggaggaggcagtga

SEQ ID NO: 23 - DNA, 1494 bp, Artificial Sequence
  Synthetic construct
gccaggccctgtatccctaagagctttggctacagctcagtagtttgtgtctgtaatgccacatactgtgactcctttgacccccctaccttccctgccctgggaaccttcagcagatatgagtcaacaagatcaggaaggaggatggagctgtcaatgggacccatccaggctaatcacacaggcacaggcctgctgctgaccctgcagccagaacagaagttccagaaagtgaagggatttggaggagccatgacagatgctgctgctctcaacatcctggccctgtcaccccctgcccagaatctgctgctgaagtcatacttctctgaagaaggaattggatataacatcatcagggtgcccatggccagctgtgacttctccatcaggacctacacctatgctgacacccctgatgatttccagctgcacaacttcagcctcccagaggaagataccaagctcaagatccctctgatacatagggcactgcagctggcccagaggcctgtgtcactcctggccagcccctggacatcacccacttggctcaagaccaatggagctgtgaatggaaagggatcactcaagggacagcctggagacatctaccaccagacctgggccagatactttgtgaagttcctggatgcctatgctgagcacaagctgcagttctgggcagtgacagctcagaatgagccttctgctggactgctgtcaggataccccttccagtgtctgggcttcacccctgaacatcagagggacttcattgccagggacctgggacctacccttgccaactcaactcaccacaatgtcaggctgctcatgctggatgaccagaggctgctgctgccccactgggccaaggtggtgctgacagacccagaagctgctaaatatgtgcatggcattgctgtgcattgctacctggacttcctggctccagccaaggccaccctgggagagacacacaggctgttccccaacaccatgctctttgcctctgagtgctgtgtgggctccaagttctgggagcagtcagtgaggctgggctcctgggataggggaatgcagtacagccacagcatcatcacaaacctcctgtaccatgtggtgggctggactgactggaacctggccctgaaccctgaaggaggacccaactgggtcagaaattttgtggactcacccatcattgtggacatcaccaaggacacattctacaagcagcccatgttctaccacctgggccacttcagcaagttcatccctgagggctcccagagggtgggactggtggcctcacagaagaatgacctggatgcagtggccctgatgcatcctgatggctctgctgtggtggttgtgctgaatagatcctctaaggatgtgcctctgaccatcaaggatcctgctgtgggcttcctggagacaatctcacctggctactccatccacacctacctgtggaggaggcagtga

SEQ ID NO: 24 - DNA, 1494 bp, Artificial Sequence
  Synthetic construct
gccaggccctgcatccctaagagctttggctacagctctgtggtgtgtgtgtgcaatgccacatactgtgactcctttgacccccccacctttcctgccctgggcacattctccagatatgagagcacaagatctgggagaaggatggagctgagcatggggcccatccaggctaatcacactggcacaggcctgctgctgaccctgcagcctgaacagaagtttcagaaagtgaagggatttggaggggccatgacagatgctgctgctctgaatatcctggccctgtcaccccctgcccagaatctgctgctgaagagctacttttcagaagaaggaattggatataatatcatcagagtgcccatggccagctgtgacttttccatcagaacctacacctatgcagacacccctgatgattttcagctgcacaattttagcctgcctgaggaagataccaagctgaagatacccctgattcacagggccctgcagctggcccagaggcctgtttcactgctggccagcccctggacatcacccacctggctgaagaccaatggagctgtgaatgggaaggggtcactgaagggacagcctggagacatctaccaccagacctgggccagatactttgtgaagtttctggatgcctatgctgagcacaagctgcagttttgggcagtgacagctcagaatgagccttcagctgggctgctgtcaggatacccctttcagtgcctgggctttacccctgaacatcagagggactttattgccagggacctgggccctaccctggccaatagcacccaccataatgtgaggttgctgatgctggatgaccagaggctgctgctgccccactgggcaaaggtggtgctgacagaccctgaagcagctaaatatgttcatggcattgctgtgcattgctacctggactttctggctcctgccaaggccaccctgggggagacacacaggctgtttcccaataccatgctgtttgcctctgagtgctgtgtgggctccaagttttgggagcagtctgtgaggctgggctcctgggatagagggatgcagtacagccacagcatcatcaccaatctgctgtaccatgtggtgggctggactgactggaatctggccctgaatcctgaaggaggacctaactgggtcaggaattttgtggacagccccatcattgtggacatcaccaaggacaccttttacaagcagcccatgttttaccacctgggccactttagcaagtttattcctgagggctcccagagagtggggctggttgccagccagaagaatgacctggatgcagtggcactgatgcatcctgatggctcagctgttgtggtggtgctgaatagatccagcaaggatgtgcctctgaccatcaaggatcctgctgtgggctttctggagacaatctcacctggctactccattcacacctacctgtggagaaggcagtga

SEQ ID NO: 25 - DNA, 1494 bp, Artificial Sequence
  Synthetic construct
gccaggccttgcatcccaaagtctttcggctacagctccgtggtgtgcgtgtgcaacgccacctattgtgactccttcgatccccctacctttcccgccctgggcacattttctagatacgagtctacacgcagcggccggagaatggagctgagcatgggccctatccaggccaatcacacaggaacaggcctgctgctgaccctgcagccagagcagaagttccagaaggtgaagggctttggcggagccatgacagatgcagccgccctgaacatcctggccctgtccccacccgcccagaatctgctgctgaagtcctacttctctgaggagggcatcggctataacatcatccgggtgcccatggccagctgcgacttttccatcagaacctacacatatgccgatacccctgacgatttccagctgcacaatttttccctgccagaggaggatacaaagctgaagatccccctgattcaccgggccctgcagctggcacagcggcccgtgagcctgctggccagcccctggacctcccctacatggctgaagaccaacggcgccgtgaatggcaagggctctctgaagggacagcctggcgacatctaccaccagacatgggccagatatttcgtgaagtttctggatgcctacgccgagcacaagctgcagttctgggccgtgacagcacagaatgagccttctgccggcctgctgagcggctatcccttccagtgcctgggctttacacctgagcaccagcgggactttatcgccagagatctgggcccaaccctggccaactccacacaccacaatgtgaggctgctgatgctggacgatcagcgcctgctgctgcctcactgggccaaggtggtgctgaccgacccagaggccgccaagtacgtgcacggcatcgccgtgcactgctatctggatttcctggcacctgcaaaggccaccctgggagagacacaccggctgttccctaacaccatgctgtttgccagcgagtgctgcgtgggctccaagttttgggagcagtccgtgaggctgggatcttgggacagaggcatgcagtactcccactctatcatcaccaatctgctgtatcacgtggtgggctggacagactggaacctggccctgaatccagagggcggccccaactgggtgagaaatttcgtggatagccccatcatcgtggacatcaccaaggatacattctacaagcagccaatgttttatcacctgggccacttctctaagtttatccctgagggcagccagagggtgggcctggtggccagccagaagaacgacctggatgccgtggccctgatgcaccctgatggctccgccgtggtggtggtgctgaatcgctctagcaaggacgtgcctctgaccatcaaggatccagccgtgggatttctggagactatttcacctggctattcaattcatacctacctgtggaggaggcagtga

SEQ ID NO: 26 - DNA, 1611 bp, Artificial Sequence
  Synthetic construct
atggagttttcaagtccttccagagaggaatgtcccaagcctttgagtagggtaagcatcatggctggcagcctcacaggattgcttctacttcaggcagtgtcgtgggcatcaggtgccaggccctgcatccctaagagctttggctacagctctgtggtgtgtgtgtgcaatgccacctactgtgacagctttgacccccccacctttcctgccctgggcaccttcagcagatatgagagcaccaggtctgggaggaggatggagctgagcatggggcccatccaggctaatcacactggcactggcctgctgctgaccctgcagcctgagcagaagttccagaaagtaaagggctttggaggggccatgactgatgctgctgctctgaacatcctggccctgagcccccctgcccagaatctgctgctgaagagctacttctctgaggagggcattggctataacatcatcagggtgcccatggccagctgtgacttcagcatcaggacctacacctatgctgacacccctgatgatttccagctgcacaacttcagcctgcctgaggaggataccaagctgaagatcccactgatccacagggctctgcagctggcccagaggcctgtgagcctgctggccagcccctggaccagccccacttggctgaagaccaatggggctgtgaatgggaaggggagcctgaagggacagcctggagacatctaccaccagacctgggccagatactttgtgaagttcctggatgcctatgctgagcacaagctgcagttctgggctgtgactgctcagaatgagccttctgctgggctgctgtctggctaccccttccaatgcctgggcttcacccctgagcatcagagggacttcattgccagggacctgggccctaccctggccaacagcactcaccataatgttaggctgctgatgctggatgaccagaggctgctgctgccccactgggctaaggtggtgctgactgaccctgaggctgctaaatatgtgcatggcattgctgtgcattgctacctggactttctggctcctgccaaggccaccctgggggagacccacaggctgttccccaacaccatgctgtttgcctctgagtgctgtgtgggcagcaagttctgggagcagtctgtgaggctgggcagctgggatagggggatgcagtacagccacagcatcatcaccaacctgctgtaccatgtggtgggctggactgactggaacctggccctgaaccctgagggaggacctaactgggtcagaaactttgtggacagccccatcattgtggacatcaccaaggacaccttttacaagcagcccatgttctaccacctgggccacttcagcaagttcatccctgagggcagccagagagtggggctggtggccagccagaagaatgacctggatgctgtggctctgatgcatcctgatggctctgctgtggtggtggtgctgaacaggagctctaaggatgtgcctctgaccatcaaggatcctgctgtgggcttcctggagaccatcagccctggctacagcatccacacctacctgtggaggaggcagtga

SEQ ID NO: 27 - DNA, 1611 bp, Artificial Sequence
  Synethtic construct
atggagttttcaagtccttccagagaggaatgtcccaagcctttgagtagggtaagcatcatggctggcagcctcacaggattgcttctacttcaggcagtgtcgtgggcatcaggtgccaggccctgtatccctaagagctttggctacagctcagtagtttgtgtctgtaatgccacatactgtgactcctttgacccccctaccttccctgccctgggaaccttcagcagatatgagtcaacaagatcaggaaggaggatggagctgtcaatgggacccatccaggctaatcacacaggcacaggcctgctgctgaccctgcagccagaacagaagttccagaaagtgaagggatttggaggagccatgacagatgctgctgctctcaacatcctggccctgtcaccccctgcccagaatctgctgctgaagtcatacttctctgaagaaggaattggatataacatcatcagggtgcccatggccagctgtgacttctccatcaggacctacacctatgctgacacccctgatgatttccagctgcacaacttcagcctcccagaggaagataccaagctcaagatccctctgatacatagggcactgcagctggcccagaggcctgtgtcactcctggccagcccctggacatcacccacttggctcaagaccaatggagctgtgaatggaaagggatcactcaagggacagcctggagacatctaccaccagacctgggccagatactttgtgaagttcctggatgcctatgctgagcacaagctgcagttctgggcagtgacagctcagaatgagccttctgctggactgctgtcaggataccccttccagtgtctgggcttcacccctgaacatcagagggacttcattgccagggacctgggacctacccttgccaactcaactcaccacaatgtcaggctgctcatgctggatgaccagaggctgctgctgccccactgggccaaggtggtgctgacagacccagaagctgctaaatatgtgcatggcattgctgtgcattgctacctggacttcctggctccagccaaggccaccctgggagagacacacaggctgttccccaacaccatgctctttgcctctgagtgctgtgtgggctccaagttctgggagcagtcagtgaggctgggctcctgggataggggaatgcagtacagccacagcatcatcacaaacctcctgtaccatgtggtgggctggactgactggaacctggccctgaaccctgaaggaggacccaactgggtcagaaattttgtggactcacccatcattgtggacatcaccaaggacacattctacaagcagcccatgttctaccacctgggccacttcagcaagttcatccctgagggctcccagagggtgggactggtggcctcacagaagaatgacctggatgcagtggccctgatgcatcctgatggctctgctgtggtggttgtgctgaatagatcctctaaggatgtgcctctgaccatcaaggatcctgctgtgggcttcctggagacaatctcacctggctactccatccacacctacctgtggaggaggcagtga

SEQ ID NO: 28 - DNA, 1611 bp, Artificial Sequence
  Synthetic construct
atggagttttcaagtccttccagagaggaatgtcccaagcctttgagtagggtaagcatcatggctggcagcctcacaggattgcttctacttcaggcagtgtcgtgggcatcaggtgccaggccctgcatccctaagagctttggctacagctctgtggtgtgtgtgtgcaatgccacatactgtgactcctttgacccccccacctttcctgccctgggcacattctccagatatgagagcacaagatctgggagaaggatggagctgagcatggggcccatccaggctaatcacactggcacaggcctgctgctgaccctgcagcctgaacagaagtttcagaaagtgaagggatttggaggggccatgacagatgctgctgctctgaatatcctggccctgtcaccccctgcccagaatctgctgctgaagagctacttttcagaagaaggaattggatataatatcatcagagtgcccatggccagctgtgacttttccatcagaacctacacctatgcagacacccctgatgattttcagctgcacaattttagcctgcctgaggaagataccaagctgaagatacccctgattcacagggccctgcagctggcccagaggcctgtttcactgctggccagcccctggacatcacccacctggctgaagaccaatggagctgtgaatgggaaggggtcactgaagggacagcctggagacatctaccaccagacctgggccagatactttgtgaagtttctggatgcctatgctgagcacaagctgcagttttgggcagtgacagctcagaatgagccttcagctgggctgctgtcaggatacccctttcagtgcctgggctttacccctgaacatcagagggactttattgccagggacctgggccctaccctggccaatagcacccaccataatgtgaggttgctgatgctggatgaccagaggctgctgctgccccactgggcaaaggtggtgctgacagaccctgaagcagctaaatatgttcatggcattgctgtgcattgctacctggactttctggctcctgccaaggccaccctgggggagacacacaggctgtttcccaataccatgctgtttgcctctgagtgctgtgtgggctccaagttttgggagcagtctgtgaggctgggctcctgggatagagggatgcagtacagccacagcatcatcaccaatctgctgtaccatgtggtgggctggactgactggaatctggccctgaatcctgaaggaggacctaactgggtcaggaattttgtggacagccccatcattgtggacatcaccaaggacaccttttacaagcagcccatgttttaccacctgggccactttagcaagtttattcctgagggctcccagagagtggggctggttgccagccagaagaatgacctggatgcagtggcactgatgcatcctgatggctcagctgttgtggtggtgctgaatagatccagcaaggatgtgcctctgaccatcaaggatcctgctgtgggctttctggagacaatctcacctggctactccattcacacctacctgtggagaaggcagtga

SEQ ID NO: 29 - DNA, 1611 bp, Artificial Sequence
  Synthetic construct
atggagttttcaagtccttccagagaggaatgtcccaagcctttgagtagggtaagcatcatggctggcagcctcacaggattgcttctacttcaggcagtgtcgtgggcatcaggtgccaggccttgcatcccaaagtctttcggctacagctccgtggtgtgcgtgtgcaacgccacctattgtgactccttcgatccccctacctttcccgccctgggcacattttctagatacgagtctacacgcagcggccggagaatggagctgagcatgggccctatccaggccaatcacacaggaacaggcctgctgctgaccctgcagccagagcagaagttccagaaggtgaagggctttggcggagccatgacagatgcagccgccctgaacatcctggccctgtccccacccgcccagaatctgctgctgaagtcctacttctctgaggagggcatcggctataacatcatccgggtgcccatggccagctgcgacttttccatcagaacctacacatatgccgatacccctgacgatttccagctgcacaatttttccctgccagaggaggatacaaagctgaagatccccctgattcaccgggccctgcagctggcacagcggcccgtgagcctgctggccagcccctggacctcccctacatggctgaagaccaacggcgccgtgaatggcaagggctctctgaagggacagcctggcgacatctaccaccagacatgggccagatatttcgtgaagtttctggatgcctacgccgagcacaagctgcagttctgggccgtgacagcacagaatgagccttctgccggcctgctgagcggctatcccttccagtgcctgggctttacacctgagcaccagcgggactttatcgccagagatctgggcccaaccctggccaactccacacaccacaatgtgaggctgctgatgctggacgatcagcgcctgctgctgcctcactgggccaaggtggtgctgaccgacccagaggccgccaagtacgtgcacggcatcgccgtgcactgctatctggatttcctggcacctgcaaaggccaccctgggagagacacaccggctgttccctaacaccatgctgtttgccagcgagtgctgcgtgggctccaagttttgggagcagtccgtgaggctgggatcttgggacagaggcatgcagtactcccactctatcatcaccaatctgctgtatcacgtggtgggctggacagactggaacctggccctgaatccagagggcggccccaactgggtgagaaatttcgtggatagccccatcatcgtggacatcaccaaggatacattctacaagcagccaatgttttatcacctgggccacttctctaagtttatccctgagggcagccagagggtgggcctggtggccagccagaagaacgacctggatgccgtggccctgatgcaccctgatggctccgccgtggtggtggtgctgaatcgctctagcaaggacgtgcctctgaccatcaaggatccagccgtgggatttctggagactatttcacctggctattcaattcatacctacctgtggaggaggcagtga

SEQ ID NO: 30 - DNA, 185 bp, Artificial Sequence
  Synthetic construct
gggcgactcagatcccagccagtggacttagcccctgtttgctcctccgataactggggtgaccttggttaatattcaccagcagcctcccccgttgcccctctggatccactgcttaaatacggacgaggacagggccctgtctcctcagcttcaggcaccaccactgacctgggacagtgaat

SEQ ID NO: 31 - DNA, 418 bp, Artificial Sequence
  Synthetic construct
ggatcttgctaccagtggaacagccactaaggattctgcagtgagagcagagggccagctaagtggtactctcccagagactgtctgactcacgccaccccctccaccttggacacaggacgctgtggtttctgagccaggtacaatgactcctttcggtaagtgcagtggaagctgtacactgcccaggcaaagcgtccgggcagcgtaggcgggcgactcagatcccagccagtggacttagcccctgtttgctcctccgataactggggtgaccttggttaatattcaccagcagcctcccccgttgcccctctggatccactgcttaaatacggacgaggacagggccctgtctcctcagcttcaggcaccaccactgacctgggacagtgaatgatccccctgatctgcggcc

SEQ ID NO: 32 - DNA, 117 bp, Artificial Sequence
  Synthetic construct
ccctaaaatgggcaaacattgcaagcagcaaacagcaaacacacagccctccctgcctgctgaccttggagctggggcagaggtcagacacctctctgggcccatgccacctccaac

SEQ ID NO: 33 - DNA, 321 bp, Artificial Sequence
  Synthetic construct
aggctcagaggcacacaggagtttctgggctcaccctgcccccttccaacccctcagttcccatcctccagcagctgtttgtgtgctgcctctgaagtccacactgaacaaacttcagcctactcatgtccctaaaatgggcaaacattgcaagcagcaaacagcaaacacacagccctccctgcctgctgaccttggagctggggcagaggtcagagacctctctgggcccatgccacctccaacatccactcgaccccttggaatttcggtggagaggagcagaggttgtcctggcgtggtttaggtagtgtgagaggg

SEQ ID NO: 34 - DNA, 334 bp, Artificial Sequence
  Synthetic construct
ccctaaaatgggcaaacattgcaagcagcaaacagcaaacacacagccctccctgcctgctgaccttggagctggggcagaggtcagacacctctctgggcccatgccacctccaactggacacaggacgctgtggtttctgagccagggggcgactcagatcccagccagtggacttagcccctgtttgctcctccgataactggggtgaccttggttaatattcaccagcagcctcccccgttgcccctctggatccactgcttaaatacggacgaggacagggccctgtctcctcagcttcaggcaccaccactgacctgggacagtgaat

SEQ ID NO: 35 - DNA, 747 bp, Artificial Sequence
  Synthetic construct
aggctcagaggcacacaggagtttctgggctcaccctgcccccttccaacccctcagttcccatcctccagcagctgtttgtgtgctgcctctgaagtccacactgaacaaacttcagcctactcatgtccctaaaatgggcaaacattgcaagcagcaaacagcaaacacacagccctccctgcctgctgaccttggagctggggcagaggtcagagacctctctgggcccatgccacctccaacatccactcgaccccttggaatttcggtggagaggagcagaggttgtcctggcgtggtttaggtagtgtgagaggggtacccggggatcttgctaccagtggaacagccactaaggattctgcagtgagagcagagggccagctaagtggtactctcccagagactgtctgactcacgccaccccctccaccttggacacaggacgctgtggtttctgagccaggtacaatgactcctttcggtaagtgcagtggaagctgtacactgcccaggcaaagcgtccgggcagcgtaggcgggcgactcagatcccagccagtggacttagcccctgtttgctcctccgataactggggtgaccttggttaatattcaccagcagcctcccccgttgcccctctggatccactgcttaaatacggacgaggacagggccctgtctcctcagcttcaggcaccaccactgacctgggacagtgaatgatccccctgatctgcggcc

SEQ ID NO: 36 - protein, 736 aa, adeno-associated virus 3B
MAADGYLPDWLEDNLSEGIREWWALKPGVPQPKANQQHQDNRRGLVLPGYKYLGPGNGLDKGEPVNEADAAALEHDKAYDQQLKAGDNPYLKYNHADAEFQERLQEDTSFGGNLGRAVFQAKKRILEPLGLVEEAAKTAPGKKRPVDQSPQEPDSSSGVGKSGKQPARKRLNFGQTGDSESVPDPQPLGEPPAAPTSLGSNTMASGGGAPMADNNEGADGVGNSSGNWHCDSQWLGDRVITTSTRTWALPTYNNHLYKQISSQSGASNDNHYFGYSTPWGYFDFNRFHCHFSPRDWQRLINNNWGFRPKKLSFKLFNIQVKEVTQNDGTTTIANNLTSTVQVFTDSEYQLPYVLGSAHQGCLPPFPADVFMVPQYGYLTLNNGSQAVGRSSFYCLEYFPSQMLRTGNNFQFSYTFEDVPFHSSYAHSQSLDRLMNPLIDQYLYYLNRTQGTTSGTTNQSRLLFSQAGPQSMSLQARNWLPGPCYRQQRLSKTANDNNNSNFPWTAASKYHLNGRDSLVNPGPAMASHKDDEEKFFPMHGNLIFGKEGTTASNAELDNVMITDEEEIRTTNPVATEQYGTVANNLQSSNTAPTTRTVNDQGALPGMVWQDRDVYLQGPIWAKIPHTDGHFHPSPLMGGFGLKHPPPQIMIKNTPVPANPPTTFSPAKFASFITQYSTGQVSVEIEWELQKENSKRWNPEIQYTSNYNKSVNVDFTVDTNGVYSEPRPIGTRYLTRNL

SEQ ID NO: 37 - protein, 736 aa, Artificial Sequence
  Synthetic capsid protein
MAADGYLPDWLEDNLSEGIREWWALKPGAPKPKANQQKQDDGRGLVLPGYKYLGPFNGLDKGEPVNAADAAALEHDKAYDQQLQAGDNPYLRYNHADAEFQERLQEDTSFGGNLGRAVFQAKKRVLEPLGLVEEGAKTAPGKKRPVDQSPQEPDSSSGVGKSGKQPARKRLNFGQTGDSESVPDPQPLGEPPAAPTSLGSNTMASGGGAPMADNNEGADGVGNSSGNWHCDSQWLGDRVITTSTRTWALPTYNNHLYKQISSQSGASNDNHYFGYSTPWGYFDFNRFHCHFSPRDWQRLINNNWGFRPKKLSFKLFNIQVKEVTQNDGTTTIANNLTSTVQVFTDSEYQLPYVLGSAHQGCLPPFPADVFMVPQYGYLTLNNGSQAVGRSSFYCLEYFPSQMLRTGNNFQFSYTFEDVPFHSSYAHSQSLDRLMNPLIDQYLYYLNRTQGTTSGTTNQSRLLFSQAGPQSMSLQARNWLPGPCYRQQRLSKTANDNNNSNFPWTAASKYHLNGRDSLVNPGPAMASHKDDEEKFFPMHGNLIFGKEGTTASNAELDNVMITDEEEIRTTNPVATEQYGTVANNLQSSNTAPTTRTVNDQGALPGMVWQDRDVYLQGPIWAKIPHTDGHFHPSPLMGGFGLKHPPPQIMIKNTPVPANPPTTFSPAKFASFITQYSTGQVSVEIEWELQKENSKRWNPEIQYTSNYNKSVNVDFTVDTNGVYSEPRPIGTRYLTRNL

SEQ ID NO: 38 - protein, 736 aa, Artificial Sequence
  Synthetic capsid protein
MAADGYLPDWLEDNLSEGIREWWALQPGAPKPKANQQHQDNARGLVLPGYKYLGPGNGLDKGEPVNAADAAALEHDKAYDQQLKAGDNPYLKYNHADAEFQERLKEDTSFGGNLGRAVFQAKKRLLEPLGLVEEAAKTAPGKKRPVDQSPQEPDSSSGVGKSGKQPARKRLNFGQTGDSESVPDPQPLGEPPAAPTSLGSNTMASGGGAPMADNNEGADGVGNSSGNWHCDSQWLGDRVITTSTRTWALPTYNNHLYKQISSQSGASNDNHYFGYSTPWGYFDFNRFHCHFSPRDWQRLINNNWGFRPKKLSFKLFNIQVKEVTQNDGTTTIANNLTSTVQVFTDSEYQLPYVLGSAHQGCLPPFPADVFMVPQYGYLTLNNGSQAVGRSSFYCLEYFPSQMLRTGNNFQFSYTFEDVPFHSSYAHSQSLDRLMNPLIDQYLYYLNRTQGTTSGTTNQSRLLFSQAGPQSMSLQARNWLPGPCYRQQRLSKTANDNNNSNFPWTAASKYHLNGRDSLVNPGPAMASHKDDEEKFFPMHGNLIFGKEGTTASNAELDNVMITDEEEIRTTNPVATEQYGTVANNLQSSNTAPTTRTVNDQGALPGMVWQDRDVYLQGPIWAKIPHTDGHFHPSPLMGGFGLKHPPPQIMIKNTPVPANPPTTFSPAKFASFITQYSTGQVSVEIEWELQKENSKRWNPEIQYTSNYNKSVNVDFTVDTNGVYSEPRPIGTRYLTRPL

SEQ ID NO: 39 - protein, 736 aa, adeno-associated virus 9
MAADGYLPDWLEDNLSEGIREWWALKPGAPQPKANQQHQDNARGLVLPGYKYLGPGNGLDKGEPVNAADAAALEHDKAYDQQLKAGDNPYLKYNHADAEFQERLKEDTSFGGNLGRAVFQAKKRLLEPLGLVEEAAKTAPGKKRPVEQSPQEPDSSAGIGKSGAQPAKKRLNFGQTGDTESVPDPQPIGEPPAAPSGVGSLTMASGGGAPVADNNEGADGVGSSSGNWHCDSQWLGDRVITTSTRTWALPTYNNHLYKQISNSTSGGSSNDNAYFGYSTPWGYFDFNRFHCHFSPRDWQRLINNNWGFRPKRLNFKLFNIQVKEVTDNNGVKTIANNLTSTVQVFTDSDYQLPYVLGSAHEGCLPPFPADVFMIPQYGYLTLNDGSQAVGRSSFYCLEYFPSQMLRTGNNFQFSYEFENVPFHSSYAHSQSLDRLMNPLIDQYLYYLSKTINGSGQNQQTLKFSVAGPSNMAVQGRNYIPGPSYRQQRVSTTVTQNNNSEFAWPGASSWALNGRNSLMNPGPAMASHKEGEDRFFPLSGSLIFGKQGTGRDNVDADKVMITNEEEIKTTNPVATESYGQVATNHQSAQAQAQTGWVQNQGILPGMVWQDRDVYLQGPIWAKIPHTDGNFHPSPLMGGFGMKHPPPQILIKNTPVPADPPTAFNKDKLNSFITQYSTGQVSVEIEWELQKENSKRWNPEIQYTSNYYKSNNVEFAVNTEGVYSEPRPIGTRYLTRNL

SEQ ID NO: 40 - DNA, 1611 bp, Homo sapiens
atggagttttcaagtccttccagagaggaatgtcccaagcctttgagtagggtaagcatcatggctggcagcctcacaggattgcttctacttcaggcagtgtcgtgggcatcaggtgcccgcccctgcatccctaaaagcttcggctacagctcggtggtgtgtgtctgcaatgccacatactgtgactcctttgaccccccgacctttcctgcccttggtaccttcagccgctatgagagtacacgcagtgggcgacggatggagctgagtatggggcccatccaggctaatcacacgggcacaggcctgctactgaccctgcagccagaacagaagttccagaaagtgaagggatttggaggggccatgacagatgctgctgctctcaacatccttgccctgtcaccccctgcccaaaatttgctacttaaatcgtacttctctgaagaaggaatcggatataacatcatccgggtacccatggccagctgtgacttctccatccgcacctacacctatgcagacacccctgatgatttccagttgcacaacttcagcctcccagaggaagataccaagctcaagatacccctgattcaccgagccctgcagttggcccagcgtcccgtttcactccttgccagcccctggacatcacccacttggctcaagaccaatggagcggtgaatgggaaggggtcactcaagggacagcccggagacatctaccaccagacctgggccagatactttgtgaagttcctggatgcctatgctgagcacaagttacagttctgggcagtgacagctgaaaatgagccttctgctgggctgttgagtggataccccttccagtgcctgggcttcacccctgaacatcagcgagacttcattgcccgtgacctaggtcctaccctcgccaacagtactcaccacaatgtccgcctactcatgctggatgaccaacgcttgctgctgccccactgggcaaaggtggtactgacagacccagaagcagctaaatatgttcatggcattgctgtacattggtacctggactttctggctccagccaaagccaccctaggggagacacaccgcctgttccccaacaccatgctctttgcctcagaggcctgtgtgggctccaagttctgggagcagagtgtgcggctaggctcctgggatcgagggatgcagtacagccacagcatcatcacgaacctcctgtaccatgtggtcggctggaccgactggaaccttgccctgaaccccgaaggaggacccaattgggtgcgtaactttgtcgacagtcccatcattgtagacatcaccaaggacacgttttacaaacagcccatgttctaccaccttggccacttcagcaagttcattcctgagggctcccagagagtggggctggttgccagtcagaagaacgacctggacgcagtggcactgatgcatcccgatggctctgctgttgtggtcgtgctaaaccgctcctctaaggatgtgcctcttaccatcaaggatcctgctgtgggcttcctggagacaatctcacctggctactccattcacacctacctgtggcgtcgccagtga

SEQ ID NO: 41 - protein, 536 aa, Artificial Sequence
  Synthetic GCase protein
MEFSSPSREECPKPLSRVSIMAGSLTGLLLLQAVSWASGARPCIPKSFGYSSVVCVCNATYCDSFDPPTFPALGTFSRYESTRSGRRMELSMGPIQANHTGTGLLLTLQPEQKFQKVKGFGGAMTDAAALNILALSPPAQNLLLKSYFSEEGIGYNIIRVPMASCDFSIRTYTYADTPDDFQLHNFSLPEEDTKLKIPLIHRALQLAQRPVSLLASPWTSPTWLKTNGAVNGKGSLKGQPGDIYHQTWARYFVKFLDAYAEHKLQFWAVTAQNEPSAGLLSGYPFQCLGFTPEHQRDFIARDLGPTLANSTHHNVRLLMLDDQRLLLPHWAKVVLTDPEAAKYVHGIAVHWYLDFLAPAKATLGETHRLFPNTMLFASEACVGSKFWEQSVRLGSWDRGMQYSHSIITNLLYHVVGWTDWNLALNPEGGPNWVRNFVDSPIIVDITKDTFYKQPMFYHLGHFSKFIPEGSQRVGLVASQKNDLDAVALMHPDGSAVVVVLNRSSKDVPLTIKDPAVGFLETISPGYSIHTYLWRRQ

SEQ ID NO: 42 - protein, 536 aa, Artificial Sequence
  Synthetic GCase protein
MEFSSPSREECPKPLSRVSIMAGSLTGLLLLQAVSWASGARPCIPKSFGYSSVVCVCNATYCDSFDPPTFPALGTFSRYESTRSGRRMELSMGPIQANHTGTGLLLTLQPEQKFQKVKGFGGAMTDAAALNILALSPPAQNLLLKSYFSEEGIGYNIIRVPMASCDFSIRTYTYADTPDDFQLHNFSLPEEDTKLKIPLIHRALQLAQRPVSLLASPWTSPTWLKTNGAVNGKGSLKGQPGDIYHQTWARYFVKFLDAYAEHKLQFWAVTAENEPSAGLLSGYPFQCLGFTPEHQRDFIARDLGPTLANSTHHNVRLLMLDDQRLLLPHWAKVVLTDPEAAKYVHGIAVHCYLDFLAPAKATLGETHRLFPNTMLFASECCVGSKFWEQSVRLGSWDRGMQYSHSIITNLLYHVVGWTDWNLALNPEGGPNWVRNFVDSPIIVDITKDTFYKQPMFYHLGHFSKFIPEGSQRVGLVASQKNDLDAVALMHPDGSAVVVVLNRSSKDVPLTIKDPAVGFLETISPGYSIHTYLWRRQ

SEQ ID NO: 43 - protein, 536 aa, Artificial Sequence
  Synthetic GCase protein
MEFSSPSREECPKPLSRVSIMAGSLTGLLLLQAVSWASGARPCIPKSFGYSSVVCVCNATYCDSFDPPTFPALGTFSRYESTRSGRRMELSMGPIQANHTGTGLLLTLQPEQKFQKVKGFGGAMTDAAALNILALSPPAQNLLLKSYFSEEGIGYNIIRVPMASCDFSIRTYTYADTPDDFQLHNFSLPEEDTKLKIPLIHRALQLAQRPVSLLASPWTSPTWLKTNGAVNGKGSLKGQPGDIYHQTWARYFVKFLDAYAEHKLQFWAVTAQNEPSAGLLSGYPFQCLGFTPEHQRDFIARDLGPTLANSTHHNVRLLMLDDQRLLLPHWAKVVLTDPEAAKYVHGIAVHCYLDFLAPAKATLGETHRLFPNTMLFASECCVGSKFWEQSVRLGSWDRGMQYSHSIITNLLYHVVGWTDWNLALNPEGGPNWVRNFVDSPIIVDITKDTFYKQPMFYHLGHFSKFIPEGSQRVGLVASQKNDLDAVALMHPDGSAVVVVLNRSSKDVPLTIKDPAVGFLETISPGYSIHTYLWRRQ

SEQ ID NO: 44 - protein, 497 aa, Artificial Sequence
  Synthetic GCase protein
ARPCIPKSFGYSSVVCVCNATYCDSFDPPTFPALGTFSRYESTRSGRRMELSMGPIQANHTGTGLLLTLQPEQKFQKVKGFGGAMTDAAALNILALSPPAQNLLLKSYFSEEGIGYNIIRVPMASCDFSIRTYTYADTPDDFQLHNFSLPEEDTKLKIPLIHRALQLAQRPVSLLASPWTSPTWLKTNGAVNGKGSLKGQPGDIYHQTWARYFVKFLDAYAEHKLQFWAVTAQNEPSAGLLSGYPFQCLGFTPEHQRDFIARDLGPTLANSTHHNVRLLMLDDQRLLLPHWAKVVLTDPEAAKYVHGIAVHWYLDFLAPAKATLGETHRLFPNTMLFASEACVGSKFWEQSVRLGSWDRGMQYSHSIITNLLYHVVGWTDWNLALNPEGGPNWVRNFVDSPIIVDITKDTFYKQPMFYHLGHFSKFIPEGSQRVGLVASQKNDLDAVALMHPDGSAVVVVLNRSSKDVPLTIKDPAVGFLETISPGYSIHTYLWRRQ

SEQ ID NO: 45 - protein, 497 aa, Artificial Sequence
  Synthetic GCase protein
ARPCIPKSFGYSSVVCVCNATYCDSFDPPTFPALGTFSRYESTRSGRRMELSMGPIQANHTGTGLLLTLQPEQKFQKVKGFGGAMTDAAALNILALSPPAQNLLLKSYFSEEGIGYNIIRVPMASCDFSIRTYTYADTPDDFQLHNFSLPEEDTKLKIPLIHRALQLAQRPVSLLASPWTSPTWLKTNGAVNGKGSLKGQPGDIYHQTWARYFVKFLDAYAEHKLQFWAVTAENEPSAGLLSGYPFQCLGFTPEHQRDFIARDLGPTLANSTHHNVRLLMLDDQRLLLPHWAKVVLTDPEAAKYVHGIAVHCYLDFLAPAKATLGETHRLFPNTMLFASECCVGSKFWEQSVRLGSWDRGMQYSHSIITNLLYHVVGWTDWNLALNPEGGPNWVRNFVDSPIIVDITKDTFYKQPMFYHLGHFSKFIPEGSQRVGLVASQKNDLDAVALMHPDGSAVVVVLNRSSKDVPLTIKDPAVGFLETISPGYSIHTYLWRRQ

SEQ ID NO: 46 - protein, 497 aa, Artificial Sequence
  Synthetic GCase protein
ARPCIPKSFGYSSVVCVCNATYCDSFDPPTFPALGTFSRYESTRSGRRMELSMGPIQANHTGTGLLLTLQPEQKFQKVKGFGGAMTDAAALNILALSPPAQNLLLKSYFSEEGIGYNIIRVPMASCDFSIRTYTYADTPDDFQLHNFSLPEEDTKLKIPLIHRALQLAQRPVSLLASPWTSPTWLKTNGAVNGKGSLKGQPGDIYHQTWARYFVKFLDAYAEHKLQFWAVTAQNEPSAGLLSGYPFQCLGFTPEHQRDFIARDLGPTLANSTHHNVRLLMLDDQRLLLPHWAKVVLTDPEAAKYVHGIAVHCYLDFLAPAKATLGETHRLFPNTMLFASECCVGSKFWEQSVRLGSWDRGMQYSHSIITNLLYHVVGWTDWNLALNPEGGPNWVRNFVDSPIIVDITKDTFYKQPMFYHLGHFSKFIPEGSQRVGLVASQKNDLDAVALMHPDGSAVVVVLNRSSKDVPLTIKDPAVGFLETISPGYSIHTYLWRRQ

SEQ ID NO: 47 - DNA, 1611 bp, Artificial Sequence
  Synthetic construct
atggagttttcaagtccttccagagaggaatgtcccaagcctttgagtagggtaagcatcatggctggcagcctcacaggattgcttctacttcaggcagtgtcgtgggcatcaggtgccaggccctgcatccctaagagctttggctacagctctgtggtgtgtgtgtgcaatgccacctactgtgacagctttgacccccccacctttcctgccctgggcaccttcagcagatatgagagcaccaggtctgggaggaggatggagctgagcatggggcccatccaggctaatcacactggcactggcctgctgctgaccctgcagcctgagcagaagttccagaaagtaaagggctttggaggggccatgactgatgctgctgctctgaacatcctggccctgagcccccctgcccagaatctgctgctgaagagctacttctctgaggagggcattggctataacatcatcagggtgcccatggccagctgtgacttcagcatcaggacctacacctatgctgacacccctgatgatttccagctgcacaacttcagcctgcctgaggaggataccaagctgaagatcccactgatccacagggctctgcagctggcccagaggcctgtgagcctgctggccagcccctggaccagccccacttggctgaagaccaatggggctgtgaatgggaaggggagcctgaagggacagcctggagacatctaccaccagacctgggccagatactttgtgaagttcctggatgcctatgctgagaacaagctgcagttctgggctgtgactgctgagaatgagccttctgctgggctgctgtctggctaccccttccaatgcctgggcttcacccctgagcatcagagggacttcattgccagggacctgggccctaccctggccaacagcactcaccataatgttaggctgctgatgctggatgaccagaggctgctgctgccccactgggctaaggtggtgctgactgaccctgaggctgctaaatatgtgcatggcattgctgtgcattggtacctggactttctggctcctgccaaggccaccctgggggagacccacaggctgttccccaacaccatgctgtttgcctctgaggcctgtgtgggcagcaagttctgggagcagtctgtgaggctgggcagctgggatagggggatgcagtacagccacagcatcatcaccaacctgctgtaccatgtggtgggctggactgactggaacctggccctgaaccctgagggaggacctaactgggtcagaaactttgtggacagccccatcattgtggacatcaccaaggacaccttttacaagcagcccatgttctaccacctgggccacttcagcaagttcatccctgagggcagccagagagtggggctggtggccagccagaagaatgacctggatgctgtggctctgatgcatcctgatggctctgctgtggtggtggtgctgaacaggagctctaaggatgtgcctctgaccatcaaggatcctgctgtgggcttcctggagaccatcagccctggctacagcatccacacctacctgtggaggaggcagtga

SEQ ID NO: 48 - DNA, 1611 bp, Artificial Sequence
  Synthetic construct
atggagttttcaagtccttccagagaggaatgtcccaagcctttgagtagggtaagcatcatggctggcagcctcacaggattgcttctacttcaggcagtgtcgtgggcatcaggtgccaggccctgcatccctaagagctttggctacagctctgtggtgtgtgtgtgcaatgccacctactgtgacagctttgacccccccacctttcctgccctgggcaccttcagcagatatgagagcaccaggtctgggaggaggatggagctgagcatggggcccatccaggctaatcacactggcactggcctgctgctgaccctgcagcctgagcagaagttccagaaagtaaagggctttggaggggccatgactgatgctgctgctctgaacatcctggccctgagcccccctgcccagaatctgctgctgaagagctacttctctgaggagggcattggctataacatcatcagggtgcccatggccagctgtgacttcagcatcaggacctacacctatgctgacacccctgatgatttccagctgcacaacttcagcctgcctgaggaggataccaagctgaagatcccactgatccacagggctctgcagctggcccagaggcctgtgagcctgctggccagcccctggaccagccccacttggctgaagaccaatggggctgtgaatgggaaggggagcctgaagggacagcctggagacatctaccaccagacctgggccagatactttgtgaagttcctggatgcctatgctgagcacaagctgcagttctgggctgtgactgctgagaatgagccttctgctgggctgctgtctggctaccccttccaatgcctgggcttcacccctgagcatcagagggacttcattgccagggacctgggccctaccctggccaacagcactcacaacaatgttaggctgctgatgctggatgaccagaggctgctgctgccccactgggctaaggtggtgctgactgaccctgaggctgctaaatatgtgcatggcattgctgtgcattggtacctggactttctggctcctgccaaggccaccctgggggagacccacaggctgttccccaacaccatgctgtttgcctctgaggcctgtgtgggcagcaagttctgggagcagtctgtgaggctgggcagctgggatagggggatgcagtacagccacagcatcatcaccaacctgctgtaccatgtggtgggctggactgactggaacctggccctgaaccctgagggaggacctaactgggtcagaaactttgtggacagccccatcattgtggacatcaccaaggacaccttttacaagcagcccatgttctaccacctgggccacttcagcaagttcatccctgagggcagccagagagtggggctggtggccagccagaagaatgacctggatgctgtggctctgatgcatcctgatggctctgctgtggtggtggtgctgaacaggagctctaaggatgtgcctctgaccatcaaggatcctgctgtgggcttcctggagaccatcagccctggctacagcatccacacctacctgtggaggaggcagtga

SEQ ID NO: 49 - DNA, 1611 bp, Artificial Sequence
  Synthetic construct
atggagttttcaagtccttccagagaggaatgtcccaagcctttgagtagggtaagcatcatggctggcagcctcacaggattgcttctacttcaggcagtgtcgtgggcatcaggtgccaggccctgcatccctaagagctttggctacagctctgtggtgtgtgtgtgcaatgccacctactgtgacagctttgacccccccacctttcctgccctgggcaccttcagcagatatgagagcaccaggtctgggaggaggatggagctgagcatggggcccatccaggctaatcacactggcactggcctgctgctgaccctgcagcctgagcagaagttccagaaagtaaagggctttggaggggccatgactgatgctgctgctctgaacatcctggccctgagcccccctgcccagaatctgctgctgaagagctacttctctgaggagggcattggctataacatcatcagggtgcccatggccagctgtgacttcagcatcaggacctacacctatgctgacacccctgatgatttccagctgcacaacttcagcctgcctgaggaggataccaagctgaagatcccactgatccacagggctctgcagctggcccagaggcctgtgagcctgctggccagcccctggaccagccccacttggctgaagaccaatggggctgtgaatgggaaggggagcctgaagggacagcctggagacatctaccaccagacctgggccagatactttgtgaagttcctggatgcctatgctgagcacaagctgcagttctgggctgtgactgctgagaatgagccttctgctgggctgctgtctggctaccccttccaatgcctgggcttcacccctgagcatcagagggacttcattgccagggacctgggccctaccctggccaacagcactcaccataatgttaggctgctgatgctggatgaccagaggctgctgctgccccactgggctaaggtggtgctgactgaccctgaggctgctaaatatgtgcatggcattgctgtgcattggtacctggactttctggctcctgccaaggccaccctgggggagacccacaggctgttccccaacaccatgctgtttgcctctgaggcctgtgtgggcagcaagttctgggagcagtctgtgaggctgggcagctgggatagggggatgcagtacagcaagagcatcatcaccaacctgctgtaccatgtggtgggctggactgactggaacctggccctgaaccctgagggaggacctaactgggtcagaaactttgtggacagccccatcattgtggacatcaccaaggacaccttttacaagcagcccatgttctaccacctgggccacttcagcaagttcatccctgagggcagccagagagtggggctggtggccagccagaagaatgacctggatgctgtggctctgatgcatcctgatggctctgctgtggtggtggtgctgaacaggagctctaaggatgtgcctctgaccatcaaggatcctgctgtgggcttcctggagaccatcagccctggctacagcatccacacctacctgtggaggaggcagtga

SEQ ID NO: 50 - DNA, 1611 bp, Artificial Sequence
  Synthetic construct
atggagttttcaagtccttccagagaggaatgtcccaagcctttgagtagggtaagcatcatggctggcagcctcacaggattgcttctacttcaggcagtgtcgtgggcatcaggtgccaggccctgcatccctaagagctttggctacagctctgtggtgtgtgtgtgcaatgccacctactgtgacagctttgacccccccacctttcctgccctgggcaccttcagcagatatgagagcaccaggtctgggaggaggatggagctgagcatggggcccatccaggctaatcacactggcactggcctgctgctgaccctgcagcctgagcagaagttccagaaagtaaagggctttggaggggccatgactgatgctgctgctctgaacatcctggccctgagcccccctgcccagaatctgctgctgaagagctacttctctgaggagggcattggctataacatcatcagggtgcccatggccagctgtgacttcagcatcaggacctacacctatgctgacacccctgatgatttccagctgcacaacttcagcctgcctgaggaggataccaagctgaagatcccactgatccacagggctctgcagctggcccagaggcctgtgagcctgctggccagcccctggaccagccccacttggctgaagaccaatggggctgtgaatgggaaggggagcctgaagggacagcctggagacatctaccaccagacctgggccagatactttgtgaagttcctggatgcctatgctgagcacaagctgcagttctgggctgtgactgctgagaatgagccttctgctgggctgctgtctggctaccccttccaatgcctgggcttcacccctgagcatcagagggacttcattgccagggacctgggccctaccctggccaacagcactcaccataatgttaggctgctgatgctggatgaccagaggctgctgctgccccactgggctaaggtggtgctgactgaccctgaggctgctaaatatgtgcatggcattgctgtgcattggtacctggactttctggctcctgccaaggccaccctgggggagacccacaggctgttccccaacaccatgctgtttgcctctgaggcctgtgtgggcagcaagttctgggagcagtctgtgaggctgggcagctgggatagggggatgcagtacagccacagcatcatcaccaacctgctgtaccatgtggtgggctggactgactggaacctggccctgaaccctgagggaggacctaactgggtcagaaactttgtggacagccccatcattgtggacatcaccaaggacaccttttacaagcagcccatgttctaccacctgggccacttcagcaagttcatccctgagggcagccagagagtggggctggtggccagccagaagaatgacctggatgctgtggctctgatgaagcctgatggctctgctgtggtggtggtgctgaacaggagctctaaggatgtgcctctgaccatcaaggatcctgctgtgggcttcctggagaccatcagccctggctacagcatccacacctacctgtggaggaggcagtga

SEQ ID NO: 51 - DNA, 1611 bp, Artificial Sequence
  Synthetic construct
atggagttttcaagtccttccagagaggaatgtcccaagcctttgagtagggtaagcatcatggctggcagcctcacaggattgcttctacttcaggcagtgtcgtgggcatcaggtgccaggccctgcatccctaagagctttggctacagctctgtggtgtgtgtgtgcaatgccacctactgtgacagctttgacccccccacctttcctgccctgggcaccttcagcagatatgagagcaccaggtctgggaggaggatggagctgagcatggggcccatccaggctaatcacactggcactggcctgctgctgaccctgcagcctgagcagaagttccagaaagtaaagggctttggaggggccatgactgatgctgctgctctgaacatcctggccctgagcccccctgcccagaatctgctgctgaagagctacttctctgaggagggcattggctataacatcatcagggtgcccatggccagctgtgacttcagcatcaggacctacacctatgctgacacccctgatgatttccagctgcacaacttcagcctgcctgaggaggataccaagctgaagatcccactgatccacagggctctgcagctggcccagaggcctgtgagcctgctggccagcccctggaccagccccacttggctgaagaccaatggggctgtgaatgggaaggggagcctgaagggacagcctggagacatctaccaccagacctgggccagatactttgtgaagttcctggatgcctatgctgagcacaagctgcagttctgggctgtgactgctgagaatgagccttctgctgggctgctgtctggctaccccttccaatgcctgggcttcacccctgagcatcagagggacttcattgccagggacctgggccctaccctggccaacagcactcaccataatgttaggctgctgatgctggatgaccagaggctgctgctgccccactgggctaaggtggtgctgactgaccctgaggctgctaaatatgtgcatggcattgctgtgcattggtacctggactttctggctcctgccaaggccaccctgggggagacccacaggctgttccccaacaccatgctgtttgcctctgaggcctgtgtgggcagcaagttctgggagcagtctgtgaggctgggcagctgggatagggggatgcagtacagccacagcatcatcaccaacctgctgtaccatgtggtgggctggactgactggaacctggccctgaaccctgagggaggacctaactgggtcagaaactttgtggacagccccatcattgtggacatcaccaaggacaccttttacaagcagcccatgttctaccacctgggccacttcagcaagttcatccctgagggcagccagagagtggggctggtggccagccagaagaatgacctggatgctgtggctctgatgcatcctgatggctctgctgtggtggtggtgctgaacaggagctctaaggatgtgcctctgaccatcaaggatcctgctgtgggcttcctggagaccatcagccctggctacagcatccacacctacctgtggaacaggcagtga

SEQ ID NO: 52 - DNA, 1611 bp, Artificial Sequence
  Synthetic construct
atggagttttcaagtccttccagagaggaatgtcccaagcctttgagtagggtaagcatcatggctggcagcctcacaggattgcttctacttcaggcagtgtcgtgggcatcaggtgccaggccctgcatccctaagagctttggctacagctctgtggtgtgtgtgtgcaatgccacctactgtgacagctttgacccccccacctttcctgccctgggcaccttcagcagatatgagagcaccaggtctgggaggaggatggagctgagcatggggcccatccaggctaatcacactggcactggcctgctgctgaccctgcagcctgagcagaagttccagaaagtaaagggctttggaggggccatgactgatgctgctgctctgaacatcctggccctgagcccccctgcccagaatctgctgctgaagagctacttctctgaggagggcattggctataacatcatcagggtgcccatggccagctgtgacttcagcatcaggacctacacctatgctgacacccctgatgatttccagctgctgaacttcagcctgcctgaggaggataccaagctgaagatcccactgatccacagggctctgcagctggcccagaggcctgtgagcctgctggccagcccctggaccagccccacttggctgaagaccaatggggctgtgaatgggaaggggagcctgaagggacagcctggagacatctaccaccagacctgggccagatactttgtgaagttcctggatgcctatgctgagcacaagctgcagttctgggctgtgactgctgagaatgagccttctgctgggctgctgtctggctaccccttccaatgcctgggcttcacccctgagcatcagagggacttcattgccagggacctgggccctaccctggccaacagcactcaccataatgttaggctgctgatgctggatgaccagaggctgctgctgccccactgggctaaggtggtgctgactgaccctgaggctgctaaatatgtgcatggcattgctgtgcattggtacctggactttctggctcctgccaaggccaccctgggggagacccacaggctgttccccaacaccatgctgtttgcctctgaggcctgtgtgggcagcaagttctgggagcagtctgtgaggctgggcagctgggatagggggatgcagtacagccacagcatcatcaccaacctgctgtaccatgtggtgggctggactgactggaacctggccctgaaccctgagggaggacctaactgggtcagaaactttgtggacagccccatcattgtggacatcaccaaggacaccttttacaagcagcccatgttctaccacctgggccacttcagcaagttcatccctgagggcagccagagagtggggctggtggccagccagaagaatgacctggatgctgtggctctgatgcatcctgatggctctgctgtggtggtggtgctgaacaggagctctaaggatgtgcctctgaccatcaaggatcctgctgtgggcttcctggagaccatcagccctggctacagcatccacacctacctgtggaggaggcagtga

SEQ ID NO: 53 - DNA, 1611 bp, Artificial Sequence
  Synthetic construct
atggagttttcaagtccttccagagaggaatgtcccaagcctttgagtagggtaagcatcatggctggcagcctcacaggattgcttctacttcaggcagtgtcgtgggcatcaggtgccaggccctgcatccctaagagctttggctacagctctgtggtgtgtgtgtgcaatgccacctactgtgacagctttgacccccccacctttcctgccctgggcaccttcagcagatatgagagcaccaggtctgggaggaggatggagctgagcatggggcccatccaggctaatcacactggcactggcctgctgctgaccctgcagcctgagcagaagttccagaaagtaaagggctttggaggggccatgactgatgctgctgctctgaacatcctggccctgagcccccctgcccagaatctgctgctgaagagctacttctctgaggagggcattggctataacatcatcagggtgcccatggccagctgtgacttcagcatcaggacctacacctatgctgacacccctgatgatttccagctgctgaacttcagcctgcctgaggaggataccaagctgaagatcccactgatccacagggctctgcagctggcccagaggcctgtgagcctgctggccagcccctggaccagccccacttggctgaagaccaatggggctgtgaatgggaaggggagcctgaagggacagcctggagacatctaccaccagacctgggccagatactttgtgaagttcctggatgcctatgctgagcacaagctgcagttctgggctgtgactgctgagaatgagccttctgctgggctgctgtctggctaccccttccaatgcctgggcttcacccctgagcatcagagggacttcattgccagggacctgggccctaccctggccaacagcactcaccataatgttaggctgctgatgctggatgaccagaggctgctgctgccccactgggctaaggtggtgctgactgaccctgaggctgctaaatatgtgcatggcattgctgtgcattggtacctggactttctggctcctgccaacgccaccctgggggagacccacaggctgttccccaacaccatgctgtttgcctctgaggcctgtgtgggcagcaagttctgggagcagtctgtgaggctgggcagctgggatagggggatgcagtacagccacagcatcatcaccaacctgctgtaccatgtggtgggctggactgactggaacctggccctgaaccctgagggaggacctaactgggtcagaaactttgtggacagccccatcattgtggacatcaccaaggacaccttttacaagcagcccatgttctaccacctgggccacttcagcaagttcatccctgagggcagccagagagtggggctggtggccagccagaagaatgacctggatgctgtggctctgatgcatcctgatggctctgctgtggtggtggtgctgaacaggagctctaaggatgtgcctctgaccatcaaggatcctgctgtgggcttcctggagaccatcagccctggctacagcatccacacctacctgtggaggaggcagtga

SEQ ID NO: 54 - DNA, 1611 bp, Artificial Sequence
  Synthetic construct
atggagttttcaagtccttccagagaggaatgtcccaagcctttgagtagggtaagcatcatggctggcagcctcacaggattgcttctacttcaggcagtgtcgtgggcatcaggtgccaggccctgcatccctaagagctttggctacagctctgtggtgtgtgtgtgcaatgccacctactgtgacagctttgacccccccacctttcctgccctgggcaccttcagcagatatgagagcaccaggtctgggaggaggatggagctgagcatggggcccatccaggctaatcacactggcactggcctgctgctgaccctgcagcctgagcagaagttccagaaagtaaagggctttggaggggccatgactgatgctgctgctctgaacatcctggccctgagcccccctgcccagaatctgctgctgaagagctacttctctgaggagggcattggctataacatcatcagggtgcccatggccagctgtgacttcagcatcaggacctacacctatgctgacacccctgatgatttccagctgcacaacttcagcctgcctgaggaggataccaagctgaagatcccactgatccacagggctctgcagctggcccagaggcctgtgagcctgctggccagcccctggaccagccccacttggctgaagaccaatggggctgtgaatgggaaggggagcctgaagggacagcctggagacatctaccaccagacctgggccagatactttgtgaagttcctggatgcctatgctgagcacaagctgcagttctgggctgtgactgctgagaatgagccttctgctgggctgctgtctggctaccccttccaatgcctgggcttcacccctgagcatcagagggacttcattgccagggacctgggccctaccctggccaacagcactcaccataatgttaggctgctgatgctggatgaccagaggctgctgctgccccactgggctaaggtggtgctgactgaccctgaggctgctaaatatgtgcatggcattgctgtgcattggtacctggactttctggctcctgccaaggccaccctgggggagacccacaggctgttccccaacaccatgctgtttgcctctgaggcctgtgtgggcagcaagttctgggagcagtctgtgaggctgggcagctgggatagggggatgcagtacagccacagcatcatcaccaacctgctgtaccatgtggtgggctggactgactggaacctggccctgaaccctgagggaggacctaactgggtcagaaactttgtggacagccccatcattgtggacatcaccaaggacaccttttacaagcagcccatgttctaccacctgggccacttcagcaagttcatccctgagggcagccagagagtggggctggtggccagccagaagaattgcctggatgctgtggctctgatgcatcctgatggctctgctgtggtggtggtgctgaacaggtgctctaaggatgtgcctctgaccatcaaggatcctgctgtgggcttcctggagaccatcagccctggctacagcatccacacctacctgtggaggaggcagtga

SEQ ID NO: 55 - DNA, 1611 bp, Artificial Sequence
  Synthetic construct
atggagttttcaagtccttccagagaggaatgtcccaagcctttgagtagggtaagcatcatggctggcagcctcacaggattgcttctacttcaggcagtgtcgtgggcatcaggtgccaggccctgcatccctaagagctttggctacagctctgtggtgtgtgtgtgcaatgccacctactgtgacagctttgacccccccacctttcctgccctgggcaccttcagcagatatgagagcaccaggtctgggaggaggatggagctgagcatggggcccatccaggctaatcacactggcactggcctgctgctgaccctgcagcctgagcagaagttccagaaagtaaagggctttggaggggccatgactgatgctgctgctctgaacatcctggccctgagcccccctgcccagaatctgctgctgaagagctacttctctgaggagggcattggctataacatcatcagggtgcccatggccagctgtgacttcagcatcaggacctacacctatgctgacacccctgatgatttccagctgcacaacttcagcctgcctgaggaggataccaagctgaagatcccactgatccacagggctctgcagctggcccagaggcctgtgagcctgctggccagcccctggaccagccccacttggctgaagaccaatggggctgtgaatgggaaggggagcctgaagggacagcctggagacatctaccaccagacctgggccagatactttgtgaagttcctggatgcctatgctgagcacaagctgcagttctgggctgtgactgctgagaatgagccttctgctgggctgctgtctggctaccccttccaatgcctgggcttcacccctgagcatcagagggacttcattgccagggacctgggccctaccctggccaacagcactcaccataatgttaggctgctgatgctggatgaccagaggctgctgctgccccactgggctaaggtggtgctgactgaccctgaggctgctaaatatgtgcatggcattgctgtgcattggtacctggactttctggctcctgccaaggccaccctgggggagacccacaggctgttccccaacaccatgctgtttgcctctgaggcctgtgtgggcagcaagttctgggagcagtctgtgaggctgggcagctgggatagggggatgcagtacagccacagcatcatcaccaacctgctgtaccatgtggtgggctggactgactggaacctggccctgaaccctgagggaggacctaactgggtcagaaactttgtggacagccccatcattgtggacatcaccaaggacaccttttacaagcagcccatgttctaccacctgggccacttcagcaagttcatccctgagggcagccagagagtggggctggtggccagccagaagaatgacctggatgctgtggctctgatgcatcctgatggctgcgctgtggtggtggtgctgaacaggagctctaaggatgtgcctctgaccatcaaggatcctgctgtgggcttcctggagaccatcagccctggctacagcatccacacctacctgtggtgcaggcagtga

SEQ ID NO: 56 - DNA, 1611 bp, Artificial Sequence
  Synthetic construct
atggagttttcaagtccttccagagaggaatgtcccaagcctttgagtagggtaagcatcatggctggcagcctcacaggattgcttctacttcaggcagtgtcgtgggcatcaggtgccaggccctgcatccctaagagctttggctacagctctgtggtgtgtgtgtgcaatgccacctactgtgacagctttgacccccccacctttcctgccctgggcaccttcagcagatatgagagcaccaggtctgggaggaggatggagctgagcatggggcccatccaggctaatcacactggcactggcctgctgctgaccctgcagcctgagcagaagttccagaaagtaaagggctttggaggggccatgactgatgctgctgctctgaacatcctggccctgagcccccctgcccagaatctgctgctgaagagctacttctctgaggagggcattggctataacatcatcagggtgcccatggccagctgtgacttcagcatcaggacctacacctatgctgacacccctgatgatttccagctgcacaacttcagcctgcctgaggaggataccaagctgaagatcccactgatccacagggctctgcagctggcccagaggcctgtgagcctgctggccagcccctggaccagccccacttggctgaagaccaatggggctgtgaatgggaaggggagcctgaagggacagcctggagacatctaccaccagacctgggccagatactttgtgaagttcctggatgcctatgctgagcacaagctgcagttctgggctgtgactgctgagaatgagccttctgctgggctgctgtctggctaccccttccaatgcctgggcttcacccctgagcatcagagggacttcattgccagggacctgggccctaccctggccaacagcactcaccataatgttaggctgctgatgctggatgaccagaggctgctgctgccccactgggctaaggtggtgctgactgaccctgaggctgctaaatatgtgcatggcattgctgtgcattggtacctggactttctggctcctgccaaggccaccctgggggagacccacaggctgttccccaacaccatgctgtttgcctctgaggcctgtgtgggcagcaagttctgggagcagtctgtgaggctgggcagctgggatagggggatgcagtacagccacagcatctgcaccaacctgctgtaccatgtggtgggctggactgactggaacctggccctgaaccctgagggaggacctaactgggtcagaaactttgtggacagccccatcattgtggacatcaccaaggacaccttttacaagcagcccatgttctaccacctgggccacttcagcaagttcatccctgagggcagccagagagtggggctggtggccagccagaagaatgacctgtgcgctgtggctctgatgcatcctgatggctctgctgtggtggtggtgctgaacaggagctctaaggatgtgcctctgaccatcaaggatcctgctgtgggcttcctggagaccatcagccctggctacagcatccacacctacctgtggaggaggcagtga

SEQ ID NO: 57 - DNA, 66 bp, Simian virus 40
gtaaatataaaatttttaagtgtataatgtgttaaactactgattctaattgtttctctcttttag

SEQ ID NO: 58 - DNA, 208 bp, Bos taurus
ctgtgccttctagttgccagccatctgttgtttgcccctcccccgtgccttccttgaccctggaaggtgccactcccactgtcctttcctaataaaatgaggaaattgcatcgcattgtctgagtaggtgtcattctattctggggggtggggtggggcaggacagcaagggggaggattgggaagacaatagcaggcatgctgggga

SEQ ID NO: 59 - DNA, 1494 bp, Artificial Sequence
  Synthetic construct
gccaggccctgcatccctaagagctttggctacagctctgtggtgtgtgtgtgcaatgccacctactgtgacagctttgacccccccacctttcctgccctgggcaccttcagcagatatgagagcaccaggtctgggaggaggatggagctgagcatggggcccatccaggctaatcacactggcactggcctgctgctgaccctgcagcctgagcagaagttccagaaagtaaagggctttggaggggccatgactgatgctgctgctctgaacatcctggccctgagcccccctgcccagaatctgctgctgaagagctacttctctgaggagggcattggctataacatcatcagggtgcccatggccagctgtgacttcagcatcaggacctacacctatgctgacacccctgatgatttccagctgcacaacttcagcctgcctgaggaggataccaagctgaagatcccactgatccacagggctctgcagctggcccagaggcctgtgagcctgctggccagcccctggaccagccccacttggctgaagaccaatggggctgtgaatgggaaggggagcctgaagggacagcctggagacatctaccaccagacctgggccagatactttgtgaagttcctggatgcctatgctgagcacaagctgcagttctgggctgtgactgctgagaatgagccttctgctgggctgctgtctggctaccccttccaatgcctgggcttcacccctgagcatcagagggacttcattgccagggacctgggccctaccctggccaacagcactcaccataatgttaggctgctgatgctggatgaccagaggctgctgctgccccactgggctaaggtggtgctgactgaccctgaggctgctaaatatgtgcatggcattgctgtgcattggtacctggactttctggctcctgccaaggccaccctgggggagacccacaggctgttccccaacaccatgctgtttgcctctgaggcctgtgtgggcagcaagttctgggagcagtctgtgaggctgggcagctgggatagggggatgcagtacagccacagcatcatcaccaacctgctgtaccatgtggtgggctggactgactggaacctggccctgaaccctgagggaggacctaactgggtcagaaactttgtggacagccccatcattgtggacatcaccaaggacaccttttacaagcagcccatgttctaccacctgggccacttcagcaagttcatccctgagggcagccagagagtggggctggtggccagccagaagaatgacctggatgctgtggctctgatgcatcctgatggctctgctgtggtggtggtgctgaacaggagctctaaggatgtgcctctgaccatcaaggatcctgctgtgggcttcctggagaccatcagccctggctacagcatccacacctacctgtggaggaggcagtga

SEQ ID NO: 60 - DNA, 1611 bp, Artificial Sequence
  Synthetic construct
atggagttttcaagtccttccagagaggaatgtcccaagcctttgagtagggtaagcatcatggctggcagcctcacaggattgcttctacttcaggcagtgtcgtgggcatcaggtgccaggccctgcatccctaagagctttggctacagctctgtggtgtgtgtgtgcaatgccacctactgtgacagctttgacccccccacctttcctgccctgggcaccttcagcagatatgagagcaccaggtctgggaggaggatggagctgagcatggggcccatccaggctaatcacactggcactggcctgctgctgaccctgcagcctgagcagaagttccagaaagtaaagggctttggaggggccatgactgatgctgctgctctgaacatcctggccctgagcccccctgcccagaatctgctgctgaagagctacttctctgaggagggcattggctataacatcatcagggtgcccatggccagctgtgacttcagcatcaggacctacacctatgctgacacccctgatgatttccagctgcacaacttcagcctgcctgaggaggataccaagctgaagatcccactgatccacagggctctgcagctggcccagaggcctgtgagcctgctggccagcccctggaccagccccacttggctgaagaccaatggggctgtgaatgggaaggggagcctgaagggacagcctggagacatctaccaccagacctgggccagatactttgtgaagttcctggatgcctatgctgagcacaagctgcagttctgggctgtgactgctgagaatgagccttctgctgggctgctgtctggctaccccttccaatgcctgggcttcacccctgagcatcagagggacttcattgccagggacctgggccctaccctggccaacagcactcaccataatgttaggctgctgatgctggatgaccagaggctgctgctgccccactgggctaaggtggtgctgactgaccctgaggctgctaaatatgtgcatggcattgctgtgcattggtacctggactttctggctcctgccaaggccaccctgggggagacccacaggctgttccccaacaccatgctgtttgcctctgaggcctgtgtgggcagcaagttctgggagcagtctgtgaggctgggcagctgggatagggggatgcagtacagccacagcatcatcaccaacctgctgtaccatgtggtgggctggactgactggaacctggccctgaaccctgagggaggacctaactgggtcagaaactttgtggacagccccatcattgtggacatcaccaaggacaccttttacaagcagcccatgttctaccacctgggccacttcagcaagttcatccctgagggcagccagagagtggggctggtggccagccagaagaatgacctggatgctgtggctctgatgcatcctgatggctctgctgtggtggtggtgctgaacaggagctctaaggatgtgcctctgaccatcaaggatcctgctgtgggcttcctggagaccatcagccctggctacagcatccacacctacctgtggaggaggcagtga

SEQ ID NO: 61 - DNA, 588 bp, Woodchuck hepatitis virus
atcaacctctggattacaaaatttgtgaaagattgactggtattcttaactatgttgctccttttacgctatgtggatacgctgctttaatgcctttgtatcatgctattgcttcccgtatggctttcattttctcctccttgtataaatcctggttgctgtctctttatgaggagttgtggcccgttgtcaggcaacgtggcgtggtgtgcactgtgtttgctgacgcaacccccactggttggggcattgccaccacctgtcagctcctttccgggactttcgctttccccctccctattgccacggcggaactcatcgccgcctgccttgcccgctgctggacaggggctcggctgttgggcactgacaattccgtggtgttgtcggggaaatcatcgtcctttccttggctgctcgcctgtgttgccacctggattctgcgcgggacgtccttctgctacgtcccttcggccctcaatccagcggaccttccttcccgcggcctgctgccggctctgcggcctcttccgcgtcttcgccttcgccctcagacgagtcggatctccctttgggccgcctccccgc

SEQ ID NO: 62 - DNA, 245 bp, Woodchuck hepatitis virus
aatcaacctctggattacaaaatttgtgaaagattgactggtattcttaactatgttgctccttttacgctatgtggatacgctgctttaatgcctttgtatcatgctattgcttcccgtatggctttcattttctcctccttgtataaatcctggttagttcttgccacggcggaactcatcgccgcctgccttgcccgctgctggacaggggctcggctgttgggcactgacaattccgtggt

SEQ ID NO: 63 - DNA, 589 bp, Woodchuck hepatitis virus
aatcaacctctggattacaaaatttgtgaaagattgactggtattcttaactatgttgctccttttacgctatgtggatacgctgctttaatgcctttgtatcatgctattgcttcccgtatggctttcattttctcctccttgtataaatcctggttgctgtctctttatgaggagttgtggcccgttgtcaggcaacgtggcgtggtgtgcactgtgtttgctgacgcaacccccactggttggggcattgccaccacctgtcagctcctttccgggactttcgctttccccctccctattgccacggcggaactcatcgccgcctgccttgcccgctgctggacaggggctcggctgttgggcactgacaattccgtggtgttgtcggggaaatcatcgtcctttccttggctgctcgcctgtgttgccacctggattctgcgcgggacgtccttctgctacgtcccttcggccctcaatccagcggaccttccttcccgcggcctgctgccggctctgcggcctcttccgcgtcttcgccttcgccctcagacgagtcggatctccctttgggccgcctccccgc

SEQ ID NO: 64 - DNA, 1494 bp, Homo sapiens
gcccgcccctgcatccctaaaagcttcggctacagctcggtggtgtgtgtctgcaatgccacatactgtgactcctttgaccccccgacctttcctgcccttggtaccttcagccgctatgagagtacacgcagtgggcgacggatggagctgagtatggggcccatccaggctaatcacacgggcacaggcctgctactgaccctgcagccagaacagaagttccagaaagtgaagggatttggaggggccatgacagatgctgctgctctcaacatccttgccctgtcaccccctgcccaaaatttgctacttaaatcgtacttctctgaagaaggaatcggatataacatcatccgggtacccatggccagctgtgacttctccatccgcacctacacctatgcagacacccctgatgatttccagttgcacaacttcagcctcccagaggaagataccaagctcaagatacccctgattcaccgagccctgcagttggcccagcgtcccgtttcactccttgccagcccctggacatcacccacttggctcaagaccaatggagcggtgaatgggaaggggtcactcaagggacagcccggagacatctaccaccagacctgggccagatactttgtgaagttcctggatgcctatgctgagcacaagttacagttctgggcagtgacagctgaaaatgagccttctgctgggctgttgagtggataccccttccagtgcctgggcttcacccctgaacatcagcgagacttcattgcccgtgacctaggtcctaccctcgccaacagtactcaccacaatgtccgcctactcatgctggatgaccaacgcttgctgctgccccactgggcaaaggtggtactgacagacccagaagcagctaaatatgttcatggcattgctgtacattggtacctggactttctggctccagccaaagccaccctaggggagacacaccgcctgttccccaacaccatgctctttgcctcagaggcctgtgtgggctccaagttctgggagcagagtgtgcggctaggctcctgggatcgagggatgcagtacagccacagcatcatcacgaacctcctgtaccatgtggtcggctggaccgactggaaccttgccctgaaccccgaaggaggacccaattgggtgcgtaactttgtcgacagtcccatcattgtagacatcaccaaggacacgttttacaaacagcccatgttctaccaccttggccacttcagcaagttcattcctgagggctcccagagagtggggctggttgccagtcagaagaacgacctggacgcagtggcactgatgcatcccgatggctctgctgttgtggtcgtgctaaaccgctcctctaaggatgtgcctcttaccatcaaggatcctgctgtgggcttcctggagacaatctcacctggctactccattcacacctacctgtggcgtcgccagtga